European Patent Specification EP 3 941 507 B1, published September 9, 2026. Title: Recombinant CCN domain proteins and fusion proteins. Applicant: Oslo Universitetssykehus HF. The sequence listing filed with the application follows.

SEQUENCE LISTING (121 sequences)

SEQ ID NO: 1 - protein, 53 aa, Homo sapiens
CPEWSTAWGPCSTTCGLGMATRVSNQNRFCRLETQRRLCLSRPCPPSRGRSPQ

SEQ ID NO: 2 - protein, 44 aa, Homo sapiens
CIEQTTEWTACSKSCGMGFSTRVTNRNRQCEMLKQTRLCMVRPC

SEQ ID NO: 3 - protein, 44 aa, Homo sapiens
CLVQTTEWSACSKTCGMGISTRVTNDNASCRLEKQSRLCMVRPC

SEQ ID NO: 4 - protein, 44 aa, Homo sapiens
CIVQTTSWSQCSKTCGTGISTRVTNDNPECRLVKETRICEVRPC

SEQ ID NO: 5 - protein, 44 aa, Homo sapiens
CIAYTSPWSPCSTSCGLGVSTRISNVNAQCWPEQESRLCNLRPC

SEQ ID NO: 6 - protein, 44 aa, Homo sapiens
CLVQATKWTPCSRTCGMGISNRVTNENSNCEMRKEKRLCYIQPC

SEQ ID NO: 7 - protein, 53 aa, Artificial Sequence
  Modified CCN5 sequence
CAEWSTAWGPCSTTCGLGMATRVSNQNRFCRLETQRRLCLSRPCPPSRGRSPQ

SEQ ID NO: 8 - protein, 55 aa, Homo sapiens
CLVQATKWTPCSRTCGMGISNRVTNENSNCEMRKEKRLCYIQPCDSNILKTIKIP

SEQ ID NO: 9 - protein, 53 aa, Homo sapiens
CIEQTTEWTACSKSCGMGFSTRVTNRNRQCEMLKQTRLCMVRPCEQEPEQPTD

SEQ ID NO: 10 - protein, 52 aa, Homo sapiens
CLVQTTEWSACSKTCGMGISTRVTNDNASCRLEKQSRLCMVRPCEADLEENI

SEQ ID NO: 11 - protein, 52 aa, Homo sapiens
CIVQTTSWSQCSKTCGTGISTRVTNDNPECRLVKETRICEVRPCGQPVYSSL

SEQ ID NO: 12 - protein, 52 aa, Homo sapiens
CIAYTSPWSPCSTSCGLGVSTRISNVNAQCWPEQESRLCNLRPCDVDIHTLI

SEQ ID NO: 13 - protein, 229 aa, Homo sapiens
ESKYGPPCPSCPAPEFLGGPSVFLFPPKPKDTLMISRTPEVTCVVVDVSQEDPEVQFNWYVDGVEVHNAKTKPREEQFNSTYRVVSVLTVLHQDWLNGKEYKCKVSNKGLPSSIEKTISKAKGQPREPQVYTLPPSQEEMTKNQVSLTCLVKGFYPSDIAVEWESNGQPENNYKTTPPVLDSDGSFFLYSRLTVDKSRWQEGNVFSCSVMHEALHNHYTQKSLSLSLGK

SEQ ID NO: 14 - protein, 228 aa, Homo sapiens
ERKCCVECPPCPAPPVAGPSVFLFPPKPKDTLMISRTPEVTCVVVDVSHEDPEVQFNWYVDGVEVHNAKTKPREEQFNSTFRVVSVLTVVHQDWLNGKEYKCKVSNKGLPAPIEKTISKTKGQPREPQVYTLPPSREEMTKNQVSLTCLVKGFYPSDISVEWESNGQPENNYKTTPPMLDSDGSFFLYSKLTVDKSRWQQGNVFSCSVMHEALHNHYTQKSLSLSPGK

SEQ ID NO: 15 - protein, 228 aa, Artificial Sequence
  Modified Fc fragment
ESKYGPPCPPCPAPEAAGGPSVFLFPPKPKDTLMISRTPEVTCVVVDVSQEDPEVQFNWYVDGVEVHNAKTKPREEQFNSTYRVVSVLTVLHQDWLNGKEYKCKVSNKGLPSSIEKTISKAKGQPREPQVYTLPPSQEEMTKNQVSLTCLVKGFYPSDIAVEWESNGQPENNYKTTPPVLDSDGSFFLYSRLTVDKSRWQEGNVFSCSVMHEALHNHYTQKSLSLSLG

SEQ ID NO: 16 - protein, 232 aa, Artificial Sequence
  Modified Fc fragment
EPKSCDKTHTCPPCPAPELLGGPSVFLFPPKPKDTLMISRTPEVTCVVVDVSHEDPEVKFNWYVDGVEVHNAKTKPCEEQYGSTYRCVSVLTVLHQDWLNGKEYKCKVSNKALPAPIEKTISKAKGQPREPQVYTLPPSRDELTKNQVSLTCLVKGFYPSDIAVEWESNGQPENNYKTTPPVLDSDGSFFLYSKLTVDKSRWQQGNVFSCSVMHEALHNHYTQKSLSLSPGK

SEQ ID NO: 17 - protein, 231 aa, Artificial Sequence
  Modified Fc fragment
EPKSCDKTHTCPPCPAPPVAGPSVFLFPPKPKDTLMISRTPEVTCVVVDVSHEDPEVKFNWYVDGVEVHNAKTKPCEEQYGSTYRCVSVLTVLHQDWLNGKEYKCKVSNKALPAPIEKTISKAKGQPREPQVYTLPPSRDELTKNQVSLTCLVKGFYPSDIAVEWESNGQPENNYKTTPPVLDSDGSFFLYSKLTVDKSRWQQGNVFSCSVMHEALHNHYTQKSLSLSPGK

SEQ ID NO: 18 - protein, 227 aa, Artificial Sequence
  Modified Fc fragment
ESKYGPPCPPCPAPPVAGPSVFLFPPKPKDTLMISRTPEVTCVVVDVSQEDPEVQFNWYVDGVEVHNAKTKPREEQFNSTYRVVSVLTVLHQDWLNGKEYKCKVSNKGLPSSIEKTISKAKGQPREPQVYTLPPSQEEMTKNQVSLTCLVKGFYPSDIAVEWESNGQPENNYKTTPPVLDSDGSFFLYSRLTVDKSRWQEGNVFSCSVMHEALHNHYTQKSLSLSLG

SEQ ID NO: 19 - protein, 227 aa, Artificial Sequence
  Modified Fc fragment
ERKCCVECPPCPAPPVAGPSVFLFPPKPKDTLMISRTPEVTCVVVDVSQEDPEVQFNWYVDGVEVHNAKTKPREEQFNSTYRVVSVLTVLHQDWLNGKEYKCKVSNKGLPSSIEKTISKAKGQPREPQVYTLPPSQEEMTKNQVSLTCLVKGFYPSDIAVEWESNGQPENNYKTTPPVLDSDGSFFLYSRLTVDKSRWQEGNVFSCSVMHEALHNHYTQKSLSLSLG

SEQ ID NO: 20 - protein, 6 aa, Artificial Sequence
  Linker
TEGRMD

SEQ ID NO: 21 - protein, 5 aa, Artificial Sequence
  Linker
EAAAK

SEQ ID NO: 22 - protein, 40 aa, Artificial Sequence
  Linker
EAAAKEAAAKEAAAKEAAAKEAAAKEAAAKEAAAKEAAAK

SEQ ID NO: 23 - protein, 42 aa, Artificial Sequence
  Linker
TAEAAAKEAAAKEAAAKEAAAKEAAAKEAAAKEAAAKEAAAK

SEQ ID NO: 24 - protein, 43 aa, Artificial Sequence
  Linker
EAAAKEAAAKEAAAKEAAAKEAAAKEAAAKEAAAKEAAAKAAA

SEQ ID NO: 25 - protein, 45 aa, Artificial Sequence
  Linker
TAEAAAKEAAAKEAAAKEAAAKEAAAKEAAAKEAAAKEAAAKAAA

SEQ ID NO: 26 - protein, 276 aa, Artificial Sequence
  Fusion protein
CPEWSTAWGPCSTTCGLGMATRVSNQNRFCRLETQRRLCLSRPCEAAAKERKCCVECPPCPAPPVAGPSVFLFPPKPKDTLMISRTPEVTCVVVDVSQEDPEVQFNWYVDGVEVHNAKTKPREEQFNSTYRVVSVLTVLHQDWLNGKEYKCKVSNKGLPSSIEKTISKAKGQPREPQVYTLPPSQEEMTKNQVSLTCLVKGFYPSDIAVEWESNGQPENNYKTTPPVLDSDGSFFLYSRLTVDKSRWQEGNVFSCSVMHEALHNHYTQKSLSLSLG

SEQ ID NO: 27 - protein, 276 aa, Artificial Sequence
  Fusion protein
CAEWSTAWGPCSTTCGLGMATRVSNQNRFCRLETQRRLCLSRPCEAAAKERKCCVECPPCPAPPVAGPSVFLFPPKPKDTLMISRTPEVTCVVVDVSQEDPEVQFNWYVDGVEVHNAKTKPREEQFNSTYRVVSVLTVLHQDWLNGKEYKCKVSNKGLPSSIEKTISKAKGQPREPQVYTLPPSQEEMTKNQVSLTCLVKGFYPSDIAVEWESNGQPENNYKTTPPVLDSDGSFFLYSRLTVDKSRWQEGNVFSCSVMHEALHNHYTQKSLSLSLG

SEQ ID NO: 28 - protein, 287 aa, Artificial Sequence
  Fusion protein
CPEWSTAWGPCSTTCGLGMATRVSNQNRFCRLETQRRLCLSRPCPPSRGRSPQTEGRMDESKYGPPCPPCPAPEAAGGPSVFLFPPKPKDTLMISRTPEVTCVVVDVSQEDPEVQFNWYVDGVEVHNAKTKPREEQFNSTYRVVSVLTVLHQDWLNGKEYKCKVSNKGLPSSIEKTISKAKGQPREPQVYTLPPSQEEMTKNQVSLTCLVKGFYPSDIAVEWESNGQPENNYKTTPPVLDSDGSFFLYSRLTVDKSRWQEGNVFSCSVMHEALHNHYTQKSLSLSLG

SEQ ID NO: 29 - protein, 286 aa, Artificial Sequence
  Fusion protein
CPEWSTAWGPCSTTCGLGMATRVSNQNRFCRLETQRRLCLSRPCPPSRGRSPQTEGRMDESKYGPPCPPCPAPPVAGPSVFLFPPKPKDTLMISRTPEVTCVVVDVSQEDPEVQFNWYVDGVEVHNAKTKPREEQFNSTYRVVSVLTVLHQDWLNGKEYKCKVSNKGLPSSIEKTISKAKGQPREPQVYTLPPSQEEMTKNQVSLTCLVKGFYPSDIAVEWESNGQPENNYKTTPPVLDSDGSFFLYSRLTVDKSRWQEGNVFSCSVMHEALHNHYTQKSLSLSLG

SEQ ID NO: 30 - protein, 286 aa, Artificial Sequence
  Fusion protein
CPEWSTAWGPCSTTCGLGMATRVSNQNRFCRLETQRRLCLSRPCPPSRGRSPQTEGRMDERKCCVECPPCPAPPVAGPSVFLFPPKPKDTLMISRTPEVTCVVVDVSQEDPEVQFNWYVDGVEVHNAKTKPREEQFNSTYRVVSVLTVLHQDWLNGKEYKCKVSNKGLPSSIEKTISKAKGQPREPQVYTLPPSQEEMTKNQVSLTCLVKGFYPSDIAVEWESNGQPENNYKTTPPVLDSDGSFFLYSRLTVDKSRWQEGNVFSCSVMHEALHNHYTQKSLSLSLG

SEQ ID NO: 31 - protein, 325 aa, Artificial Sequence
  Fusion protein
CPEWSTAWGPCSTTCGLGMATRVSNQNRFCRLETQRRLCLSRPCPPSRGRSPQTAEAAAKEAAAKEAAAKEAAAKEAAAKEAAAKEAAAKEAAAKAAAERKCCVECPPCPAPPVAGPSVFLFPPKPKDTLMISRTPEVTCVVVDVSQEDPEVQFNWYVDGVEVHNAKTKPREEQFNSTYRVVSVLTVLHQDWLNGKEYKCKVSNKGLPSSIEKTISKAKGQPREPQVYTLPPSQEEMTKNQVSLTCLVKGFYPSDIAVEWESNGQPENNYKTTPPVLDSDGSFFLYSRLTVDKSRWQEGNVFSCSVMHEALHNHYTQKSLSLSLG

SEQ ID NO: 32 - protein, 18 aa, Homo sapiens
MKWVTFISLLFLFSSAYS

SEQ ID NO: 33 - protein, 305 aa, Artificial Sequence
  Fusion protein
MKWVTFISLLFLFSSAYSCPEWSTAWGPCSTTCGLGMATRVSNQNRFCRLETQRRLCLSRPCPPSRGRSPQTEGRMDESKYGPPCPPCPAPEAAGGPSVFLFPPKPKDTLMISRTPEVTCVVVDVSQEDPEVQFNWYVDGVEVHNAKTKPREEQFNSTYRVVSVLTVLHQDWLNGKEYKCKVSNKGLPSSIEKTISKAKGQPREPQVYTLPPSQEEMTKNQVSLTCLVKGFYPSDIAVEWESNGQPENNYKTTPPVLDSDGSFFLYSRLTVDKSRWQEGNVFSCSVMHEALHNHYTQKSLSLSLG

SEQ ID NO: 34 - DNA, 915 bp, Artificial Sequence
  Fusion protein
atgaaatgggtcacctttatctccctgctgttcctgttctcctccgcctactcttgccctgagtggtctacagcttggggcccttgctctaccacctgtggactcggcatggccaccagagtgtctaaccagaacagattctgccggctggaaacccagcggagactgtgcctgtctagaccctgtcctcctagcagaggcagatcccctcagaccgagggcagaatggacgagtctaagtacggccctccttgtcctccatgtcctgctccagaagctgctggcggcccttccgtgtttctgttccctccaaagcctaaggacaccctgatgatctctcggacccctgaagtgacctgcgtggtggtggatgtgtcccaagaggatcccgaggtgcagttcaattggtacgtggacggcgtggaagtgcacaacgccaagaccaagcctagagaggaacagttcaactccacctacagagtggtgtccgtgctgaccgtgctgcaccaggattggctgaacggcaaagagtacaagtgcaaggtgtccaacaagggcctgccttccagcatcgaaaagaccatctccaaggccaagggccagcctagggaaccccaggtttacaccctgcctccaagccaagaggaaatgaccaagaaccaggtgtccctgacctgcctggtcaagggcttctacccttccgatatcgccgtggaatgggagagcaatggccagcctgagaacaactacaagaccacacctcctgtgctggactccgacggctccttctttctgtactcccgcctgaccgtggacaagtccagatggcaagagggcaacgtgttctcctgctccgtgatgcacgaggccctgcacaatcactacacccagaagtccctgtctctgtccctgggc

SEQ ID NO: 35 - DNA, 924 bp, Artificial Sequence
  Fusion protein
gccaccatgaaatgggtcacctttatctccctgctgttcctgttctcctccgcctactcttgccctgagtggtctacagcttggggcccttgctctaccacctgtggactcggcatggccaccagagtgtctaaccagaacagattctgccggctggaaacccagcggagactgtgcctgtctagaccctgtcctcctagcagaggcagatcccctcagaccgagggcagaatggacgagtctaagtacggccctccttgtcctccatgtcctgctccagaagctgctggcggcccttccgtgtttctgttccctccaaagcctaaggacaccctgatgatctctcggacccctgaagtgacctgcgtggtggtggatgtgtcccaagaggatcccgaggtgcagttcaattggtacgtggacggcgtggaagtgcacaacgccaagaccaagcctagagaggaacagttcaactccacctacagagtggtgtccgtgctgaccgtgctgcaccaggattggctgaacggcaaagagtacaagtgcaaggtgtccaacaagggcctgccttccagcatcgaaaagaccatctccaaggccaagggccagcctagggaaccccaggtttacaccctgcctccaagccaagaggaaatgaccaagaaccaggtgtccctgacctgcctggtcaagggcttctacccttccgatatcgccgtggaatgggagagcaatggccagcctgagaacaactacaagaccacacctcctgtgctggactccgacggctccttctttctgtactcccgcctgaccgtggacaagtccagatggcaagagggcaacgtgttctcctgctccgtgatgcacgaggccctgcacaatcactacacccagaagtccctgtctctgtccctgggctaa

SEQ ID NO: 36 - DNA, 997 bp, Artificial Sequence
  Fusion protein
ggggacaagtttgtacaaaaaagcaggctatggtaccgccaccatgaaatgggtcacctttatctccctgctgttcctgttctcctccgcctactcttgccctgagtggtctacagcttggggcccttgctctaccacctgtggactcggcatggccaccagagtgtctaaccagaacagattctgccggctggaaacccagcggagactgtgcctgtctagaccctgtcctcctagcagaggcagatcccctcagaccgagggcagaatggacgagtctaagtacggccctccttgtcctccatgtcctgctccagaagctgctggcggcccttccgtgtttctgttccctccaaagcctaaggacaccctgatgatctctcggacccctgaagtgacctgcgtggtggtggatgtgtcccaagaggatcccgaggtgcagttcaattggtacgtggacggcgtggaagtgcacaacgccaagaccaagcctagagaggaacagttcaactccacctacagagtggtgtccgtgctgaccgtgctgcaccaggattggctgaacggcaaagagtacaagtgcaaggtgtccaacaagggcctgccttccagcatcgaaaagaccatctccaaggccaagggccagcctagggaaccccaggtttacaccctgcctccaagccaagaggaaatgaccaagaaccaggtgtccctgacctgcctggtcaagggcttctacccttccgatatcgccgtggaatgggagagcaatggccagcctgagaacaactacaagaccacacctcctgtgctggactccgacggctccttctttctgtactcccgcctgaccgtggacaagtccagatggcaagagggcaacgtgttctcctgctccgtgatgcacgaggccctgcacaatcactacacccagaagtccctgtctctgtccctgggctaatctagaaacccagctttcttgtacaaagtggtcccc

SEQ ID NO: 37 - protein, 44 aa, Homo sapiens
CPEWSTAWGPCSTTCGLGMATRVSNQNRFCRLETQRRLCLSRPC

SEQ ID NO: 38 - protein, 44 aa, Artificial Sequence
  Modified CCN5 sequence
CAEWSTAWGPCSTTCGLGMATRVSNQNRFCRLETQRRLCLSRPC

SEQ ID NO: 39 - protein, 44 aa, Artificial Sequence
  Linker
AEAAAKEAAAKEAAAKEAAAKEAAAKEAAAKEAAAKEAAAKAAA

SEQ ID NO: 40 - protein, 325 aa, Artificial Sequence
  Fusion protein
ESKYGPPCPPCPAPEAAGGPSVFLFPPKPKDTLMISRTPEVTCVVVDVSQEDPEVQFNWYVDGVEVHNAKTKPREEQFNSTYRVVSVLTVLHQDWLNGKEYKCKVSNKGLPSSIEKTISKAKGQPREPQVYTLPPSQEEMTKNQVSLTCLVKGFYPSDIAVEWESNGQPENNYKTTPPVLDSDGSFFLYSRLTVDKSRWQEGNVFSCSVMHEALHNHYTQKSLSLSLGAEAAAKEAAAKEAAAKEAAAKEAAAKEAAAKEAAAKEAAAKAAACPEWSTAWGPCSTTCGLGMATRVSNQNRFCRLETQRRLCLSRPCPPSRGRSPQ

SEQ ID NO: 41 - protein, 325 aa, Artificial Sequence
  Fusion protein
ESKYGPPCPPCPAPEAAGGPSVFLFPPKPKDTLMISRTPEVTCVVVDVSQEDPEVQFNWYVDGVEVHNAKTKPREEQFNSTYRVVSVLTVLHQDWLNGKEYKCKVSNKGLPSSIEKTISKAKGQPREPQVYTLPPSQEEMTKNQVSLTCLVKGFYPSDIAVEWESNGQPENNYKTTPPVLDSDGSFFLYSRLTVDKSRWQEGNVFSCSVMHEALHNHYTQKSLSLSLGAEAAAKEAAAKEAAAKEAAAKEAAAKEAAAKEAAAKEAAAKAAACAEWSTAWGPCSTTCGLGMATRVSNQNRFCRLETQRRLCLSRPCPPSRGRSPQ

SEQ ID NO: 42 - protein, 44 aa, Artificial Sequence
  Modified CCN1 sequence
CAVQTTSWSQCSKTCGTGISTRVTNDNPECRLVKETRICEVRPC

SEQ ID NO: 43 - protein, 44 aa, Artificial Sequence
  Modified CCN2 sequence
CAVQTTEWSACSKTCGMGISTRVTNDNASCRLEKQSRLCMVRPC

SEQ ID NO: 44 - protein, 44 aa, Artificial Sequence
  Modified CCN3 sequence
CAEQTTEWTACSKSCGMGFSTRVTNRNRQCEMLKQTRLCMVRPC

SEQ ID NO: 45 - protein, 44 aa, Artificial Sequence
  Modified CCN4 sequence
CAAYTSPWSPCSTSCGLGVSTRISNVNAQCWPEQESRLCNLRPC

SEQ ID NO: 46 - protein, 44 aa, Artificial Sequence
  Modified CCN6 sequence
CAVQATKWTPCSRTCGMGISNRVTNENSNCEMRKEKRLCYIQPC

SEQ ID NO: 47 - protein, 52 aa, Artificial Sequence
  Modified CCN1 sequence
CAVQTTSWSQCSKTCGTGISTRVTNDNPECRLVKETRICEVRPCGQPVYSSL

SEQ ID NO: 48 - protein, 52 aa, Artificial Sequence
  Modified CCN2 sequence
CAVQTTEWSACSKTCGMGISTRVTNDNASCRLEKQSRLCMVRPCEADLEENI

SEQ ID NO: 49 - protein, 53 aa, Artificial Sequence
  Modified CCN3 sequence
CAEQTTEWTACSKSCGMGFSTRVTNRNRQCEMLKQTRLCMVRPCEQEPEQPTD

SEQ ID NO: 50 - protein, 52 aa, Artificial Sequence
  Modified CCN4 sequence
CAAYTSPWSPCSTSCGLGVSTRISNVNAQCWPEQESRLCNLRPCDVDIHTLI

SEQ ID NO: 51 - protein, 55 aa, Artificial Sequence
  Modified CCN6 sequence
CAVQATKWTPCSRTCGMGISNRVTNENSNCEMRKEKRLCYIQPCDSNILKTIKIP

SEQ ID NO: 52 - protein, 585 aa, Homo sapiens [sequence omitted]

SEQ ID NO: 53 - protein, 679 aa, Homo sapiens
VPDKTVRWCAVSEHEATKCQSFRDHMKSVIPSDGPSVACVKKASYLDCIRAIAANEADAVTLDAGLVYDAYLAPNNLKPVVAEFYGSKEDPQTFYYAVAVVKKDSGFQMNQLRGKKSCHTGLGRSAGWNIPIGLLYCDLPEPRKPLEKAVANFFSGSCAPCADGTDFPQLCQLCPGCGCSTLNQYFGYSGAFKCLKDGAGDVAFVKHSTIFENLANKADRDQYELLCLDNTRKPVDEYKDCHLAQVPSHTVVARSMGGKEDLIWELLNQAQEHFGKDKSKEFQLFSSPHGKDLLFKDSAHGFLKVPPRMDAKMYLGYEYVTAIRNLREGTCPEAPTDECKPVKWCALSHHERLKCDEWSVNSVGKIECVSAETTEDCIAKIMNGEADAMSLDGGFVYIAGKCGLVPVLAENYNKSDNCEDTPEAGYFAIAVVKKSASDLTWDNLKGKKSCHTAVGRTAGWNIPMGLLYNKINHCRFDEFFSEGCAPGSKKDSSLCKLCMGSGLNLCEPNNKEGYYGYTGAFRCLVEKGDVAFVKHQTVPQNTGGKNPDPWAKNLNEKDYELLCLDGTRKPVEEYANCHLARAPNHAVVTRKDKEACVHKILRQQQHLFGSNVTDCSGNFCLFRSETKDLLFRDDTVCLAKLHDRNTYEKYLGEEYVKAVGNLRKCSTSSLLEACTFRRP

SEQ ID NO: 54 - protein, 232 aa, Artificial Sequence
  Modified Fc fragment
EPKSQDKTHTQPPQPAPELLGGPSVFLFPPKPKDTLMISRTPEVTCVVVDVSHEDPEVKFNWYVDGVEVHNAKTKPCEEQYGSTYRCVSVLTVLHQDWLNGKEYKCKVSNKALPAPIEKTISKAKGQPREPQVYTLPPSRDELTKNQVSLRCHVKGFYPSDIAVEWESNGQPENNYKTTKPVLDSDGSFFLYSTLTVDKSRWQQGNVFSCSVLHEALHNHYTQKSLSLSPGK

SEQ ID NO: 55 - protein, 227 aa, Artificial Sequence
  Modified Fc fragment
ERKQQVEQPPQPAPPVAGPSVFLFPPKPKDTLYITREPEVTCVVVDVSQEDPEVQFNWYVDGVEVHNAKTKPREEQFNSTYRVVSVLTVLHQDWLNGKEYKCKVSNKGLPSSIEKTISKAKGQPREPQVYTFPPSQEEMTKNQVSLRCLVKGFYPSDIAVEWESNGQPENNYKTTKPVLDSDGSFRLESRLTVDKSRWQEGNVFSCSVMHEALHNHYTQKSLSLSLG

SEQ ID NO: 56 - protein, 57 aa, Homo sapiens
CPEWSTAWGPCSTTCGLGMATRVSNQNRFCRLETQRRLCLSRPCPPSRGRSPQNSAF

SEQ ID NO: 57 - protein, 6 aa, Artificial Sequence
  Linker
IEGRMD

SEQ ID NO: 58 - protein, 291 aa, Artificial Sequence
  Fusion protein
CPEWSTAWGPCSTTCGLGMATRVSNQNRFCRLETQRRLCLSRPCPPSRGRSPQNSAFIEGRMDESKYGPPCPPCPAPEAAGGPSVFLFPPKPKDTLMISRTPEVTCVVVDVSQEDPEVQFNWYVDGVEVHNAKTKPREEQFNSTYRVVSVLTVLHQDWLNGKEYKCKVSNKGLPSSIEKTISKAKGQPREPQVYTLPPSQEEMTKNQVSLTCLVKGFYPSDIAVEWESNGQPENNYKTTPPVLDSDGSFFLYSRLTVDKSRWQEGNVFSCSVMHEALHNHYTQKSLSLSLG

SEQ ID NO: 59 - protein, 309 aa, Artificial Sequence
  Fusion protein
MKWVTFISLLFLFSSAYSCPEWSTAWGPCSTTCGLGMATRVSNQNRFCRLETQRRLCLSRPCPPSRGRSPQNSAFIEGRMDESKYGPPCPPCPAPEAAGGPSVFLFPPKPKDTLMISRTPEVTCVVVDVSQEDPEVQFNWYVDGVEVHNAKTKPREEQFNSTYRVVSVLTVLHQDWLNGKEYKCKVSNKGLPSSIEKTISKAKGQPREPQVYTLPPSQEEMTKNQVSLTCLVKGFYPSDIAVEWESNGQPENNYKTTPPVLDSDGSFFLYSRLTVDKSRWQEGNVFSCSVMHEALHNHYTQKSLSLSLG

SEQ ID NO: 60 - DNA, 936 bp, Artificial Sequence
  Fusion protein
gccaccatgaaatgggtcacctttatctccctgctgttcctgttctcctccgcctactcttgccctgagtggtctacagcttggggcccttgctctaccacctgtggactcggcatggccaccagagtgtctaaccagaacagattctgccggctggaaacccagcggagactgtgtctgtccagaccttgtcctcctagccggggcagatcccctcagaactctgcctttatcgagggcagaatggacgagtctaagtacggccctccttgtccaccatgtcctgctccagaagctgctggcggcccttccgtgtttctgttccctccaaagcctaaggacaccctgatgatctctcggacccctgaagtgacctgcgtggtggtggatgtgtcccaagaggatcccgaggtgcagttcaattggtacgtggacggcgtggaagtgcacaacgccaagaccaagcctagagaggaacagttcaactccacctacagagtggtgtccgtgctgaccgtgctgcaccaggattggctgaacggcaaagagtacaagtgcaaggtgtccaacaagggcctgccttccagcatcgaaaagaccatctccaaggccaagggccagcctagggaaccccaggtttacaccctgcctccaagccaagaggaaatgaccaagaaccaggtgtccctgacctgcctggtcaagggcttctacccttccgatatcgccgtggaatgggagagcaatggccagcctgagaacaactacaagaccacacctcctgtgctggactccgacggctccttctttctgtactcccgcctgaccgtggacaagtccagatggcaagagggcaacgtgttctcctgctccgtgatgcacgaggccctgcacaatcactacacccagaagtccctgtctctgtccctgggctaa

SEQ ID NO: 61 - DNA, 1009 bp, Artificial Sequence
  Fusion protein
ggggacaagtttgtacaaaaaagcaggctatggtaccgccaccatgaaatgggtcacctttatctccctgctgttcctgttctcctccgcctactcttgccctgagtggtctacagcttggggcccttgctctaccacctgtggactcggcatggccaccagagtgtctaaccagaacagattctgccggctggaaacccagcggagactgtgtctgtccagaccttgtcctcctagccggggcagatcccctcagaactctgcctttatcgagggcagaatggacgagtctaagtacggccctccttgtccaccatgtcctgctccagaagctgctggcggcccttccgtgtttctgttccctccaaagcctaaggacaccctgatgatctctcggacccctgaagtgacctgcgtggtggtggatgtgtcccaagaggatcccgaggtgcagttcaattggtacgtggacggcgtggaagtgcacaacgccaagaccaagcctagagaggaacagttcaactccacctacagagtggtgtccgtgctgaccgtgctgcaccaggattggctgaacggcaaagagtacaagtgcaaggtgtccaacaagggcctgccttccagcatcgaaaagaccatctccaaggccaagggccagcctagggaaccccaggtttacaccctgcctccaagccaagaggaaatgaccaagaaccaggtgtccctgacctgcctggtcaagggcttctacccttccgatatcgccgtggaatgggagagcaatggccagcctgagaacaactacaagaccacacctcctgtgctggactccgacggctccttctttctgtactcccgcctgaccgtggacaagtccagatggcaagagggcaacgtgttctcctgctccgtgatgcacgaggccctgcacaatcactacacccagaagtccctgtctctgtccctgggctaatctagaaacccagctttcttgtacaaagtggtcccc

SEQ ID NO: 62 - protein, 56 aa, Artificial Sequence
  Modified CCN5 sequence
CPEWSTAWGPCSTTCGLGMATRVSNQNRFCRLETQRRLCLSRPCPPSRGRSLQNSA

SEQ ID NO: 63 - protein, 4 aa, Artificial Sequence
  Linker
GRMD

SEQ ID NO: 64 - protein, 306 aa, Artificial Sequence
  Fusion protein
MKWVTFISLLFLFSSAYSCPEWSTAWGPCSTTCGLGMATRVSNQNRFCRLETQRRLCLSRPCPPSRGRSLQNSAGRMDESKYGPPCPPCPAPEAAGGPSVFLFPPKPKDTLMISRTPEVTCVVVDVSQEDPEVQFNWYVDGVEVHNAKTKPREEQFNSTYRVVSVLTVLHQDWLNGKEYKCKVSNKGLPSSIEKTISKAKGQPREPQVYTLPPSQEEMTKNQVSLTCLVKGFYPSDIAVEWESNGQPENNYKTTPPVLDSDGSFFLYSRLTVDKSRWQEGNVFSCSVMHEALHNHYTQKSLSLSLG

SEQ ID NO: 65 - protein, 6 aa, Artificial Sequence
  Linker
TEGRMD

SEQ ID NO: 66 - protein, 305 aa, Artificial Sequence; identical to SEQ ID NO: 33
  Fusion protein

SEQ ID NO: 67 - protein, 8 aa, Artificial Sequence
  Linker
TAEAAAKA

SEQ ID NO: 68 - protein, 307 aa, Artificial Sequence
  Fusion protein
MKWVTFISLLFLFSSAYSCPEWSTAWGPCSTTCGLGMATRVSNQNRFCRLETQRRLCLSRPCPPSRGRSPQTAEAAAKAESKYGPPCPPCPAPEAAGGPSVFLFPPKPKDTLMISRTPEVTCVVVDVSQEDPEVQFNWYVDGVEVHNAKTKPREEQFNSTYRVVSVLTVLHQDWLNGKEYKCKVSNKGLPSSIEKTISKAKGQPREPQVYTLPPSQEEMTKNQVSLTCLVKGFYPSDIAVEWESNGQPENNYKTTPPVLDSDGSFFLYSRLTVDKSRWQEGNVFSCSVMHEALHNHYTQKSLSLSLG

SEQ ID NO: 69 - protein, 304 aa, Artificial Sequence
  Fusion protein
MKWVTFISLLFLFSSAYSCPEWSTAWGPCSTTCGLGMATRVSNQNRFCRLETQRRLCLSRPCPPSRGRSPQTEGRMDERKCCVECPPCPAPPVAGPSVFLFPPKPKDTLMISRTPEVTCVVVDVSQEDPEVQFNWYVDGVEVHNAKTKPREEQFNSTYRVVSVLTVLHQDWLNGKEYKCKVSNKGLPSSIEKTISKAKGQPREPQVYTLPPSQEEMTKNQVSLTCLVKGFYPSDIAVEWESNGQPENNYKTTPPVLDSDGSFFLYSRLTVDKSRWQEGNVFSCSVMHEALHNHYTQKSLSLSLG

SEQ ID NO: 70 - protein, 294 aa, Artificial Sequence
  Fusion protein
MKWVTFISLLFLFSSAYSCAEWSTAWGPCSTTCGLGMATRVSNQNRFCRLETQRRLCLSRPCEAAAKERKCCVECPPCPAPPVAGPSVFLFPPKPKDTLMISRTPEVTCVVVDVSQEDPEVQFNWYVDGVEVHNAKTKPREEQFNSTYRVVSVLTVLHQDWLNGKEYKCKVSNKGLPSSIEKTISKAKGQPREPQVYTLPPSQEEMTKNQVSLTCLVKGFYPSDIAVEWESNGQPENNYKTTPPVLDSDGSFFLYSRLTVDKSRWQEGNVFSCSVMHEALHNHYTQKSLSLSLG

SEQ ID NO: 71 - DNA, 891 bp, Artificial Sequence
  Fusion protein
gccaccatgaaatgggtcacctttatctccctgctgttcctgttctcctccgcctactcttgcgccgagtggtctacagcttggggcccttgttctaccacctgtggcctcggcatggccaccagagtgtccaaccagaacagattctgccggctggaaacccagcggagactgtgtttgtccagaccttgcgaggccgctgccaaagaaagaaagtgctgcgtggaatgccctccttgtcctgctcctcctgtggctggcccttccgtgtttctgttccctccaaagcctaaggacaccctgatgatctctcggacccctgaagtgacctgcgtggtggtggatgtgtcccaagaggatcccgaggtgcagttcaattggtacgtggacggcgtggaagtgcacaacgccaagaccaagcctagagaggaacagttcaactccacctacagagtggtgtccgtgctgaccgtgctgcaccaggattggctgaacggcaaagagtacaagtgcaaggtgtccaacaagggactgccctccagcatcgaaaagaccatctccaaggccaagggacagcccagagaaccccaggtgtacacactgcctccaagccaagaggaaatgaccaagaaccaggtgtccctgacctgcctggtcaagggcttctacccttccgatatcgccgtggaatgggagtccaatggccagcctgagaacaactacaagaccacacctccagtgctggactccgacggctccttctttctgtactcccgcctgaccgtggacaagtccagatggcaagagggcaacgtgttctcctgctccgtgatgcacgaggccctgcacaatcactacacccagaagtccctgtctctgtccctgggctaa

SEQ ID NO: 72 - DNA, 964 bp, Artificial Sequence
  Fusion protein
ggggacaagtttgtacaaaaaagcaggctatggtaccgccaccatgaaatgggtcacctttatctccctgctgttcctgttctcctccgcctactcttgcgccgagtggtctacagcttggggcccttgttctaccacctgtggcctcggcatggccaccagagtgtccaaccagaacagattctgccggctggaaacccagcggagactgtgtttgtccagaccttgcgaggccgctgccaaagaaagaaagtgctgcgtggaatgccctccttgtcctgctcctcctgtggctggcccttccgtgtttctgttccctccaaagcctaaggacaccctgatgatctctcggacccctgaagtgacctgcgtggtggtggatgtgtcccaagaggatcccgaggtgcagttcaattggtacgtggacggcgtggaagtgcacaacgccaagaccaagcctagagaggaacagttcaactccacctacagagtggtgtccgtgctgaccgtgctgcaccaggattggctgaacggcaaagagtacaagtgcaaggtgtccaacaagggactgccctccagcatcgaaaagaccatctccaaggccaagggacagcccagagaaccccaggtgtacacactgcctccaagccaagaggaaatgaccaagaaccaggtgtccctgacctgcctggtcaagggcttctacccttccgatatcgccgtggaatgggagtccaatggccagcctgagaacaactacaagaccacacctccagtgctggactccgacggctccttctttctgtactcccgcctgaccgtggacaagtccagatggcaagagggcaacgtgttctcctgctccgtgatgcacgaggccctgcacaatcactacacccagaagtccctgtctctgtccctgggctaatctagaaacccagctttcttgtacaaagtggtcccc

SEQ ID NO: 73 - protein, 276 aa, Artificial Sequence
  Fusion protein
CAEQTTEWTACSKSCGMGFSTRVTNRNRQCEMLKQTRLCMVRPCEAAAKERKCCVECPPCPAPPVAGPSVFLFPPKPKDTLMISRTPEVTCVVVDVSQEDPEVQFNWYVDGVEVHNAKTKPREEQFNSTYRVVSVLTVLHQDWLNGKEYKCKVSNKGLPSSIEKTISKAKGQPREPQVYTLPPSQEEMTKNQVSLTCLVKGFYPSDIAVEWESNGQPENNYKTTPPVLDSDGSFFLYSRLTVDKSRWQEGNVFSCSVMHEALHNHYTQKSLSLSLG

SEQ ID NO: 74 - protein, 294 aa, Artificial Sequence
  Fusion protein
MKWVTFISLLFLFSSAYSCAEQTTEWTACSKSCGMGFSTRVTNRNRQCEMLKQTRLCMVRPCEAAAKERKCCVECPPCPAPPVAGPSVFLFPPKPKDTLMISRTPEVTCVVVDVSQEDPEVQFNWYVDGVEVHNAKTKPREEQFNSTYRVVSVLTVLHQDWLNGKEYKCKVSNKGLPSSIEKTISKAKGQPREPQVYTLPPSQEEMTKNQVSLTCLVKGFYPSDIAVEWESNGQPENNYKTTPPVLDSDGSFFLYSRLTVDKSRWQEGNVFSCSVMHEALHNHYTQKSLSLSLG

SEQ ID NO: 75 - DNA, 891 bp, Artificial Sequence
  Fusion protein
gccaccatgaaatgggtcacctttatctccctgctgttcctgttctcctccgcctactcttgtgccgagcagaccacagagtggaccgcctgctctaagtcttgcggcatgggcttctccaccagagtgaccaaccggaacagacagtgcgagatgctgaagcagacccggctgtgtatggttcgaccttgcgaggccgctgccaaagaaagaaagtgctgcgtggaatgccctccttgtcctgctcctcctgtggctggcccttccgtgtttctgttccctccaaagcctaaggacaccctgatgatctctcggacccctgaagtgacctgcgtggtggtggatgtgtcccaagaggatcccgaggtgcagttcaattggtacgtggacggcgtggaagtgcacaacgccaagaccaagcctagagaggaacagttcaactccacctacagagtggtgtccgtgctgaccgtgctgcaccaggattggctgaacggcaaagagtacaagtgcaaggtgtccaacaagggcctgccttccagcatcgaaaagaccatctccaaggccaagggacagcccagagaaccccaggtgtacacactgcctccaagccaagaggaaatgaccaagaaccaggtgtccctgacctgcctggtcaagggcttctacccttccgatatcgccgtggaatgggagtccaatggccagcctgagaacaactacaagaccacacctccagtgctggactccgacggctccttctttctgtactcccgcctgaccgtggacaagtccagatggcaagagggcaacgtgttctcctgctccgtgatgcacgaggccctgcacaatcactacacccagaagtccctgtctctgtccctgggctaa

SEQ ID NO: 76 - DNA, 964 bp, Artificial Sequence
  Fusion protein
ggggacaagtttgtacaaaaaagcaggctatggtaccgccaccatgaaatgggtcacctttatctccctgctgttcctgttctcctccgcctactcttgtgccgagcagaccacagagtggaccgcctgctctaagtcttgcggcatgggcttctccaccagagtgaccaaccggaacagacagtgcgagatgctgaagcagacccggctgtgtatggttcgaccttgcgaggccgctgccaaagaaagaaagtgctgcgtggaatgccctccttgtcctgctcctcctgtggctggcccttccgtgtttctgttccctccaaagcctaaggacaccctgatgatctctcggacccctgaagtgacctgcgtggtggtggatgtgtcccaagaggatcccgaggtgcagttcaattggtacgtggacggcgtggaagtgcacaacgccaagaccaagcctagagaggaacagttcaactccacctacagagtggtgtccgtgctgaccgtgctgcaccaggattggctgaacggcaaagagtacaagtgcaaggtgtccaacaagggcctgccttccagcatcgaaaagaccatctccaaggccaagggacagcccagagaaccccaggtgtacacactgcctccaagccaagaggaaatgaccaagaaccaggtgtccctgacctgcctggtcaagggcttctacccttccgatatcgccgtggaatgggagtccaatggccagcctgagaacaactacaagaccacacctccagtgctggactccgacggctccttctttctgtactcccgcctgaccgtggacaagtccagatggcaagagggcaacgtgttctcctgctccgtgatgcacgaggccctgcacaatcactacacccagaagtccctgtctctgtccctgggctaatctagaaacccagctttcttgtacaaagtggtcccc

SEQ ID NO: 77 - protein, 343 aa, Artificial Sequence
  Fusion protein
MKWVTFISLLFLFSSAYSESKYGPPCPPCPAPEAAGGPSVFLFPPKPKDTLMISRTPEVTCVVVDVSQEDPEVQFNWYVDGVEVHNAKTKPREEQFNSTYRVVSVLTVLHQDWLNGKEYKCKVSNKGLPSSIEKTISKAKGQPREPQVYTLPPSQEEMTKNQVSLTCLVKGFYPSDIAVEWESNGQPENNYKTTPPVLDSDGSFFLYSRLTVDKSRWQEGNVFSCSVMHEALHNHYTQKSLSLSLGAEAAAKEAAAKEAAAKEAAAKEAAAKEAAAKEAAAKEAAAKAAACAEWSTAWGPCSTTCGLGMATRVSNQNRFCRLETQRRLCLSRPCPPSRGRSPQ

SEQ ID NO: 78 - DNA, 1038 bp, Artificial Sequence
  Fusion protein
gccaccatgaaatgggtcacctttatctccctgctgttcctgttctccagcgcctactccgagtctaagtacggccctccttgtcctccatgtcctgctccagaagctgctggcggcccttccgtgtttctgttccctccaaagcctaaggacaccctgatgatctctcggacccctgaagtgacctgcgtggtggtggatgtgtcccaagaggatcccgaggtgcagttcaattggtacgtggacggcgtggaagtgcacaacgccaagaccaagcctagagaggaacagttcaactccacctacagagtggtgtccgtgctgaccgtgctgcaccaggattggctgaacggcaaagagtacaagtgcaaggtgtccaacaagggcctgccttccagcatcgaaaagaccatctccaaggccaagggccagcctagggaaccccaggtttacaccctgcctccaagccaagaggaaatgaccaagaaccaggtgtccctgacctgcctggtcaagggcttctacccttccgatatcgccgtggaatgggagagcaatggccagcctgagaacaactacaagaccacacctcctgtgctggactccgacggctccttctttctgtactcccgcctgaccgtggacaagtccagatggcaagagggcaacgtgttctcctgctccgtgatgcacgaggccctgcacaatcactacacccagaagtccctgtctctgtccctgggagctgaggccgctgctaaagaagctgccgctaaagaggccgcagccaaagaggcagccgccaaagaagccgctgcaaaagaggctgctgcaaaagaagcagcagctaaagaagctgctgccaaggccgctgcttgtgccgaatggtctacagcttggggcccttgctctaccacctgtggactcggcatggccaccagagtgtctaaccagaacagattctgccggctggaaacccagcggagactgtgcctgtctagaccctgtcctcctagcagaggcagatcccctcagtga

SEQ ID NO: 79 - DNA, 1111 bp, Artificial Sequence
  Fusion protein
ggggacaagtttgtacaaaaaagcaggctatggtaccgccaccatgaaatgggtcacctttatctccctgctgttcctgttctccagcgcctactccgagtctaagtacggccctccttgtcctccatgtcctgctccagaagctgctggcggcccttccgtgtttctgttccctccaaagcctaaggacaccctgatgatctctcggacccctgaagtgacctgcgtggtggtggatgtgtcccaagaggatcccgaggtgcagttcaattggtacgtggacggcgtggaagtgcacaacgccaagaccaagcctagagaggaacagttcaactccacctacagagtggtgtccgtgctgaccgtgctgcaccaggattggctgaacggcaaagagtacaagtgcaaggtgtccaacaagggcctgccttccagcatcgaaaagaccatctccaaggccaagggccagcctagggaaccccaggtttacaccctgcctccaagccaagaggaaatgaccaagaaccaggtgtccctgacctgcctggtcaagggcttctacccttccgatatcgccgtggaatgggagagcaatggccagcctgagaacaactacaagaccacacctcctgtgctggactccgacggctccttctttctgtactcccgcctgaccgtggacaagtccagatggcaagagggcaacgtgttctcctgctccgtgatgcacgaggccctgcacaatcactacacccagaagtccctgtctctgtccctgggagctgaggccgctgctaaagaagctgccgctaaagaggccgcagccaaagaggcagccgccaaagaagccgctgcaaaagaggctgctgcaaaagaagcagcagctaaagaagctgctgccaaggccgctgcttgtgccgaatggtctacagcttggggcccttgctctaccacctgtggactcggcatggccaccagagtgtctaaccagaacagattctgccggctggaaacccagcggagactgtgcctgtctagaccctgtcctcctagcagaggcagatcccctcagtgatctagaaacccagctttcttgtacaaagtggtcccc

SEQ ID NO: 80 - protein, 311 aa, Artificial Sequence
  Fusion protein
CAEQTTEWTACSKSCGMGFSTRVTNRNRQCEMLKQTRLCMVRPCEAAAKEAAAKEAAAKEAAAKEAAAKEAAAKEAAAKEAAAKERKCCVECPPCPAPPVAGPSVFLFPPKPKDTLMISRTPEVTCVVVDVSQEDPEVQFNWYVDGVEVHNAKTKPREEQFNSTYRVVSVLTVLHQDWLNGKEYKCKVSNKGLPSSIEKTISKAKGQPREPQVYTLPPSQEEMTKNQVSLTCLVKGFYPSDIAVEWESNGQPENNYKTTPPVLDSDGSFFLYSRLTVDKSRWQEGNVFSCSVMHEALHNHYTQKSLSLSLG

SEQ ID NO: 81 - protein, 329 aa, Artificial Sequence
  Fusion protein
MKWVTFISLLFLFSSAYSCAEQTTEWTACSKSCGMGFSTRVTNRNRQCEMLKQTRLCMVRPCEAAAKEAAAKEAAAKEAAAKEAAAKEAAAKEAAAKEAAAKERKCCVECPPCPAPPVAGPSVFLFPPKPKDTLMISRTPEVTCVVVDVSQEDPEVQFNWYVDGVEVHNAKTKPREEQFNSTYRVVSVLTVLHQDWLNGKEYKCKVSNKGLPSSIEKTISKAKGQPREPQVYTLPPSQEEMTKNQVSLTCLVKGFYPSDIAVEWESNGQPENNYKTTPPVLDSDGSFFLYSRLTVDKSRWQEGNVFSCSVMHEALHNHYTQKSLSLSLG

SEQ ID NO: 82 - DNA, 996 bp, Artificial Sequence
  Fusion protein
gccaccatgaaatgggtcacctttatctccctgctgttcctgttctcctccgcctactcttgtgccgagcagaccacagagtggaccgcctgctctaagtcttgcggcatgggcttctccaccagagtgaccaaccggaacagacagtgcgagatgctgaagcagacccggctgtgtatggttcgaccttgcgaggccgctgccaaagaggctgctgctaaagaagccgccgcaaaagaggcagcagcaaaagaggctgccgccaaagaggccgcagccaaagaagcagcagctaaagaggccgctgcaaaagaacggaagtgctgcgtggaatgccctccttgtcctgctcctcctgtggctggcccttccgtgtttctgttccctccaaagcctaaggacaccctgatgatctctcggacccctgaagtgacctgcgtggtggtggatgtgtcccaagaggatcccgaggtgcagttcaattggtacgtggacggcgtggaagtgcacaacgccaagaccaagcctagagaggaacagttcaactccacctacagagtggtgtccgtgctgaccgtgctgcaccaggattggctgaacggcaaagagtacaagtgcaaggtgtccaacaagggcctgccttccagcatcgaaaagaccatctccaaggccaagggacagcccagagaaccccaggtgtacacactgcctccaagccaagaggaaatgaccaagaaccaggtgtccctgacctgcctggtcaagggcttctacccttccgatatcgccgtggaatgggagtccaatggccagcctgagaacaactacaagaccacacctccagtgctggactccgacggctccttctttctgtactcccgcctgaccgtggacaagtccagatggcaagagggcaacgtgttctcctgctccgtgatgcacgaggccctgcacaatcactacacccagaagtccctgtctctgtccctgggctaa

SEQ ID NO: 83 - DNA, 1069 bp, Artificial Sequence
  Fusion protein
ggggacaagtttgtacaaaaaagcaggctatggtaccgccaccatgaaatgggtcacctttatctccctgctgttcctgttctcctccgcctactcttgtgccgagcagaccacagagtggaccgcctgctctaagtcttgcggcatgggcttctccaccagagtgaccaaccggaacagacagtgcgagatgctgaagcagacccggctgtgtatggttcgaccttgcgaggccgctgccaaagaggctgctgctaaagaagccgccgcaaaagaggcagcagcaaaagaggctgccgccaaagaggccgcagccaaagaagcagcagctaaagaggccgctgcaaaagaacggaagtgctgcgtggaatgccctccttgtcctgctcctcctgtggctggcccttccgtgtttctgttccctccaaagcctaaggacaccctgatgatctctcggacccctgaagtgacctgcgtggtggtggatgtgtcccaagaggatcccgaggtgcagttcaattggtacgtggacggcgtggaagtgcacaacgccaagaccaagcctagagaggaacagttcaactccacctacagagtggtgtccgtgctgaccgtgctgcaccaggattggctgaacggcaaagagtacaagtgcaaggtgtccaacaagggcctgccttccagcatcgaaaagaccatctccaaggccaagggacagcccagagaaccccaggtgtacacactgcctccaagccaagaggaaatgaccaagaaccaggtgtccctgacctgcctggtcaagggcttctacccttccgatatcgccgtggaatgggagtccaatggccagcctgagaacaactacaagaccacacctccagtgctggactccgacggctccttctttctgtactcccgcctgaccgtggacaagtccagatggcaagagggcaacgtgttctcctgctccgtgatgcacgaggccctgcacaatcactacacccagaagtccctgtctctgtccctgggctaatctagaaacccagctttcttgtacaaagtggtcccc

SEQ ID NO: 84 - protein, 276 aa, Artificial Sequence
  Fusion protein
CAEQTTEWTACSKSCGMGFSTRVTNRNRQCEMLKQTRLCMVRPCEAAAKERKQQVEQPPQPAPPVAGPSVFLFPPKPKDTLYITREPEVTCVVVDVSQEDPEVQFNWYVDGVEVHNAKTKPREEQFNSTYRVVSVLTVLHQDWLNGKEYKCKVSNKGLPSSIEKTISKAKGQPREPQVYTFPPSQEEMTKNQVSLRCLVKGFYPSDIAVEWESNGQPENNYKTTKPVLDSDGSFRLESRLTVDKSRWQEGNVFSCSVMHEALHNHYTQKSLSLSLG

SEQ ID NO: 85 - protein, 294 aa, Artificial Sequence
  Fusion protein
MKWVTFISLLFLFSSAYSCAEQTTEWTACSKSCGMGFSTRVTNRNRQCEMLKQTRLCMVRPCEAAAKERKQQVEQPPQPAPPVAGPSVFLFPPKPKDTLYITREPEVTCVVVDVSQEDPEVQFNWYVDGVEVHNAKTKPREEQFNSTYRVVSVLTVLHQDWLNGKEYKCKVSNKGLPSSIEKTISKAKGQPREPQVYTFPPSQEEMTKNQVSLRCLVKGFYPSDIAVEWESNGQPENNYKTTKPVLDSDGSFRLESRLTVDKSRWQEGNVFSCSVMHEALHNHYTQKSLSLSLG

SEQ ID NO: 86 - DNA, 891 bp, Artificial Sequence
  Fusion protein
gccaccatgaaatgggtcacctttatctccctgctgttcctgttctcctccgcctactcttgtgccgagcagaccacagagtggaccgcctgctctaagtcttgcggcatgggcttctccaccagagtgaccaaccggaacagacagtgcgagatgctgaagcagacccggctgtgtatggttcgaccttgcgaggccgctgccaaagaaagaaagcagcaggtcgagcagcctcctcagcctgctcctcctgttgctggcccttccgtgtttctgttccctccaaagcctaaggacaccctgtacatcacccgcgagcctgaagtgacctgcgtggtggtggatgtgtcccaagaggatcccgaggtgcagttcaattggtacgtggacggcgtggaagtgcacaacgccaagaccaagcctagagaggaacagttcaactccacctacagagtggtgtccgtgctgaccgtgctgcaccaggattggctgaacggcaaagagtacaagtgcaaggtgtccaacaagggcctgccttccagcatcgaaaagaccatctccaaggccaagggacagcccagagaaccccaggtgtacacattccctccatctcaagaggaaatgaccaagaaccaggtgtccctgcggtgcctggtcaagggcttctacccttctgatatcgccgtggaatgggagtccaacggccagcctgagaacaactacaagaccaccaagcctgtgctggactccgacggctccttccggcttgaatctagactgaccgtggacaagtcccggtggcaagagggcaacgtgttctcctgctctgtgatgcacgaggccctgcacaaccactacacccagaagtccctgtctctgtccctgggctaa

SEQ ID NO: 87 - DNA, 964 bp, Artificial Sequence
  Fusion protein
ggggacaagtttgtacaaaaaagcaggctatggtaccgccaccatgaaatgggtcacctttatctccctgctgttcctgttctcctccgcctactcttgtgccgagcagaccacagagtggaccgcctgctctaagtcttgcggcatgggcttctccaccagagtgaccaaccggaacagacagtgcgagatgctgaagcagacccggctgtgtatggttcgaccttgcgaggccgctgccaaagaaagaaagcagcaggtcgagcagcctcctcagcctgctcctcctgttgctggcccttccgtgtttctgttccctccaaagcctaaggacaccctgtacatcacccgcgagcctgaagtgacctgcgtggtggtggatgtgtcccaagaggatcccgaggtgcagttcaattggtacgtggacggcgtggaagtgcacaacgccaagaccaagcctagagaggaacagttcaactccacctacagagtggtgtccgtgctgaccgtgctgcaccaggattggctgaacggcaaagagtacaagtgcaaggtgtccaacaagggcctgccttccagcatcgaaaagaccatctccaaggccaagggacagcccagagaaccccaggtgtacacattccctccatctcaagaggaaatgaccaagaaccaggtgtccctgcggtgcctggtcaagggcttctacccttctgatatcgccgtggaatgggagtccaacggccagcctgagaacaactacaagaccaccaagcctgtgctggactccgacggctccttccggcttgaatctagactgaccgtggacaagtcccggtggcaagagggcaacgtgttctcctgctctgtgatgcacgaggccctgcacaaccactacacccagaagtccctgtctctgtccctgggctaatctagaaacccagctttcttgtacaaagtggtcccc

SEQ ID NO: 88 - protein, 281 aa, Artificial Sequence
  Fusion protein
CAEQTTEWTACSKSCGMGFSTRVTNRNRQCEMLKQTRLCMVRPCEAAAKEPKSQDKTHTQPPQPAPELLGGPSVFLFPPKPKDTLMISRTPEVTCVVVDVSHEDPEVKFNWYVDGVEVHNAKTKPCEEQYGSTYRCVSVLTVLHQDWLNGKEYKCKVSNKALPAPIEKTISKAKGQPREPQVYTLPPSRDELTKNQVSLRCHVKGFYPSDIAVEWESNGQPENNYKTTKPVLDSDGSFFLYSTLTVDKSRWQQGNVFSCSVLHEALHNHYTQKSLSLSPGK

SEQ ID NO: 89 - protein, 299 aa, Artificial Sequence
  Fusion protein
MKWVTFISLLFLFSSAYSCAEQTTEWTACSKSCGMGFSTRVTNRNRQCEMLKQTRLCMVRPCEAAAKEPKSQDKTHTQPPQPAPELLGGPSVFLFPPKPKDTLMISRTPEVTCVVVDVSHEDPEVKFNWYVDGVEVHNAKTKPCEEQYGSTYRCVSVLTVLHQDWLNGKEYKCKVSNKALPAPIEKTISKAKGQPREPQVYTLPPSRDELTKNQVSLRCHVKGFYPSDIAVEWESNGQPENNYKTTKPVLDSDGSFFLYSTLTVDKSRWQQGNVFSCSVLHEALHNHYTQKSLSLSPGK

SEQ ID NO: 90 - DNA, 906 bp, Artificial Sequence
  Fusion protein
gccaccatgaaatgggtcacctttatctccctgctgttcctgttctcctccgcctactcttgtgccgagcagaccacagagtggaccgcctgctctaagtcttgcggcatgggcttctccaccagagtgaccaaccggaacagacagtgcgagatgctgaagcagacccggctgtgtatggttcgaccttgcgaggccgctgccaaagagcctaagagccaggacaagacccacacacagcctccacagcctgctccagaattgctcggaggcccttccgtgtttctgttccctccaaagcctaaggacaccctgatgatctctcggacccctgaagtgacctgcgtggtggtggatgtgtctcacgaggatcccgaagtgaagttcaattggtacgtggacggcgtggaagtgcacaacgccaagacaaagccctgcgaggaacagtacggctccacctacagatgcgtgtccgtgctgacagtgctgcaccaggattggctgaacggcaaagagtacaagtgcaaggtgtccaacaaggccctgcctgctcctatcgaaaagaccatctccaaggccaagggccagcctagagaaccccaggtgtacacactgccaccttctagggacgagctgaccaagaaccaggtgtccctgagatgccacgtgaagggcttctacccctccgatatcgccgtggaatgggagtctaatggacagcccgagaacaactacaagaccaccaagcctgtgctggactccgacggctccttcttcctgtactctaccctgaccgtggacaagtccagatggcagcagggcaacgtgttctcctgctctgtgctgcacgaggccctgcacaatcactacacccagaagtccctgtctctgtcccctggcaagtga

SEQ ID NO: 91 - DNA, 979 bp, Artificial Sequence
  Fusion protein
ggggacaagtttgtacaaaaaagcaggctatggtaccgccaccatgaaatgggtcacctttatctccctgctgttcctgttctcctccgcctactcttgtgccgagcagaccacagagtggaccgcctgctctaagtcttgcggcatgggcttctccaccagagtgaccaaccggaacagacagtgcgagatgctgaagcagacccggctgtgtatggttcgaccttgcgaggccgctgccaaagagcctaagagccaggacaagacccacacacagcctccacagcctgctccagaattgctcggaggcccttccgtgtttctgttccctccaaagcctaaggacaccctgatgatctctcggacccctgaagtgacctgcgtggtggtggatgtgtctcacgaggatcccgaagtgaagttcaattggtacgtggacggcgtggaagtgcacaacgccaagacaaagccctgcgaggaacagtacggctccacctacagatgcgtgtccgtgctgacagtgctgcaccaggattggctgaacggcaaagagtacaagtgcaaggtgtccaacaaggccctgcctgctcctatcgaaaagaccatctccaaggccaagggccagcctagagaaccccaggtgtacacactgccaccttctagggacgagctgaccaagaaccaggtgtccctgagatgccacgtgaagggcttctacccctccgatatcgccgtggaatgggagtctaatggacagcccgagaacaactacaagaccaccaagcctgtgctggactccgacggctccttcttcctgtactctaccctgaccgtggacaagtccagatggcagcagggcaacgtgttctcctgctctgtgctgcacgaggccctgcacaatcactacacccagaagtccctgtctctgtcccctggcaagtgatctagaaacccagctttcttgtacaaagtggtcccc

SEQ ID NO: 92 - protein, 402 aa, Artificial Sequence
  Fusion tag
GHHHHHHGSEIGTGFPFDPHYVEVLGERMHYVDVGPRDGTPVLFLHGNPTSSYVWRNIIPHVAPTHRCIAPDLIGMGKSDKPDLGYFFDDHVRFMDAFIEALGLEEVVLVIHDWGSALGFHWAKRNPERVKGIAFMEFIRPIPTWDEWPEFARETFQAFRTTDVGRKLIIDQNVFIEGTLPMGVVRPLTEVEMDHYREPFLNPVDREPLWRFPNELPIAGEPANIVALVEEYMDWLHQSPVPKLLFWGTPGVLIPPAEAARLAKSLPNCKAVDIGPGLNLLQEDNPDLIGSEIARWLSTLEISGLQDSEVNQEAKPEVKPEVKPETHINLKVSDGSSEIFFKIKKTTPLRRLMEAFAKRQGKEMDSLTFLYDGIEIQADQTPEDLDMEDNDIIEAHREQIGG

SEQ ID NO: 93 - protein, 20 aa, Artificial Sequence
  Linker
SGGSGGSGGSGGSSGGGSSG

SEQ ID NO: 94 - protein, 466 aa, Artificial Sequence
  Fusion protein
GHHHHHHGSEIGTGFPFDPHYVEVLGERMHYVDVGPRDGTPVLFLHGNPTSSYVWRNIIPHVAPTHRCIAPDLIGMGKSDKPDLGYFFDDHVRFMDAFIEALGLEEVVLVIHDWGSALGFHWAKRNPERVKGIAFMEFIRPIPTWDEWPEFARETFQAFRTTDVGRKLIIDQNVFIEGTLPMGVVRPLTEVEMDHYREPFLNPVDREPLWRFPNELPIAGEPANIVALVEEYMDWLHQSPVPKLLFWGTPGVLIPPAEAARLAKSLPNCKAVDIGPGLNLLQEDNPDLIGSEIARWLSTLEISGLQDSEVNQEAKPEVKPEVKPETHINLKVSDGSSEIFFKIKKTTPLRRLMEAFAKRQGKEMDSLTFLYDGIEIQADQTPEDLDMEDNDIIEAHREQIGGSGGSGGSGGSGGSSGGGSSGCAEQTTEWTACSKSCGMGFSTRVTNRNRQCEMLKQTRLCMVRPC

SEQ ID NO: 95 - DNA, 1461 bp, Artificial Sequence
  Fusion protein
gccaccatgaaatgggtcacctttatctccctgctgttcctgttctcctccgcctactctggccaccaccatcaccatcacggctccgagatcggaaccggctttcctttcgaccctcactacgtggaagtgctgggcgagagaatgcactatgtggacgtgggccccagagatggaacccctgtgctgtttctgcacggcaaccctacctccagctacgtgtggcggaacatcatccctcacgtggcccctacacacagatgtatcgcccctgacctgatcggcatgggcaagtctgacaagcctgacctgggctacttcttcgacgaccacgtgcggttcatggacgcctttatcgaggctctgggcctcgaagaggtggtgctggtcatccatgattggggctctgccctgggctttcactgggccaagagaaaccccgagagagtgaagggaatcgccttcatggaattcatccggcctattcctacctgggacgagtggcctgagttcgccagagagacattccaggccttcagaaccaccgacgtgggcagaaagctgatcatcgaccagaacgtgttcatcgagggcaccctgcctatgggagtcgtcagacctctgaccgaggtggaaatggaccactacagagagccctttctgaaccccgtggaccgggaacctctttggagattccctaacgagctgcctatcgctggcgagcctgccaatattgtggccctggtggaagagtacatggactggctgcatcagagccccgtgcctaagctgctgttttggggaacacccggcgtgctgattcctcctgctgaagctgctagactggccaagagcctgcctaactgcaaggccgtggatatcggccctggcctgaatctgctgcaagaggacaaccccgatctgatcggatctgagatcgcccggtggctgagcaccctggaaatcagtggactgcaggactccgaagtgaatcaagaggccaagcctgaagtgaagcccgaagtcaagcctgagacacacatcaacctgaaggtgtccgacggctccagcgagatcttcttcaagatcaagaaaaccacacctctgcggcggctgatggaagcctttgccaagagacagggcaaagagatggactccctgaccttcctgtacgacggcatcgagatccaggccgatcagacccctgaggacctggacatggaagataacgacatcattgaggcccacagagagcagatcggcggctctggtggtagcggaggttctggtggatctggtggttcttctggcggcggatcttctggctgtgctgagcagacaaccgagtggaccgcctgctctaagtcttgtggcatgggcttctccaccagagtgaccaaccggaacagacagtgcgagatgctgaagcagacccggctgtgtatggtccgaccttgctaa

SEQ ID NO: 96 - DNA, 1552 bp, Artificial Sequence
  Fusion protein
ggggacaagtttgtacaaaaaagcaggctataagcttgctgccaccatgaaatgggtcacctttatctccctgctgttcctgttctcctccgcctactctggccaccaccatcaccatcacggctccgagatcggaaccggctttcctttcgaccctcactacgtggaagtgctgggcgagagaatgcactatgtggacgtgggccccagagatggaacccctgtgctgtttctgcacggcaaccctacctccagctacgtgtggcggaacatcatccctcacgtggcccctacacacagatgtatcgcccctgacctgatcggcatgggcaagtctgacaagcctgacctgggctacttcttcgacgaccacgtgcggttcatggacgcctttatcgaggctctgggcctcgaagaggtggtgctggtcatccatgattggggctctgccctgggctttcactgggccaagagaaaccccgagagagtgaagggaatcgccttcatggaattcatccggcctattcctacctgggacgagtggcctgagttcgccagagagacattccaggccttcagaaccaccgacgtgggcagaaagctgatcatcgaccagaacgtgttcatcgagggcaccctgcctatgggagtcgtcagacctctgaccgaggtggaaatggaccactacagagagccctttctgaaccccgtggaccgggaacctctttggagattccctaacgagctgcctatcgctggcgagcctgccaatattgtggccctggtggaagagtacatggactggctgcatcagagccccgtgcctaagctgctgttttggggaacacccggcgtgctgattcctcctgctgaagctgctagactggccaagagcctgcctaactgcaaggccgtggatatcggccctggcctgaatctgctgcaagaggacaaccccgatctgatcggatctgagatcgcccggtggctgagcaccctggaaatcagtggactgcaggactccgaagtgaatcaagaggccaagcctgaagtgaagcccgaagtcaagcctgagacacacatcaacctgaaggtgtccgacggctccagcgagatcttcttcaagatcaagaaaaccacacctctgcggcggctgatggaagcctttgccaagagacagggcaaagagatggactccctgaccttcctgtacgacggcatcgagatccaggccgatcagacccctgaggacctggacatggaagataacgacatcattgaggcccacagagagcagatcggcggctctggtggtagcggaggttctggtggatctggtggttcttctggcggcggatcttctggctgtgctgagcagacaaccgagtggaccgcctgctctaagtcttgtggcatgggcttctccaccagagtgaccaaccggaacagacagtgcgagatgctgaagcagacccggctgtgtatggtccgaccttgctaaatctagagcggccgcggtaccaacccagctttcttgtacaaagtggtcccc

SEQ ID NO: 97 - protein, 634 aa, Artificial Sequence
  Fusion protein
CAEWSTAWGPCSTTCGLGMATRVSNQNRFCRLETQRRLCLSRPCEAAAKDAHKSEVAHRFKDLGEENFKALVLIAFAQYLQQCPFEDHVKLVNEVTEFAKTCVADESAENCDKSLHTLFGDKLCTVATLRETYGEMADCCAKQEPERNECFLQHKDDNPNLPRLVRPEVDVMCTAFHDNEETFLKKYLYEIARRHPYFYAPELLFFAKRYKAAFTECCQAADKAACLLPKLDELRDEGKASSAKQRLKCASLQKFGERAFKAWAVARLSQRFPKAEFAEVSKLVTDLTKVHTECCHGDLLECADDRADLAKYICENQDSISSKLKECCEKPLLEKSHCIAEVENDEMPADLPSLAADFVESKDVCKNYAEAKDVFLGMFLYEYARRHPDYSVVLLLRLAKTYETTLEKCCAAADPHECYAKVFDEFKPLVEEPQNLIKQNCELFEQLGEYKFQNALLVRYTKKVPQVSTPTLVEVSRNLGKVGSKCCKHPEAKRMPCAEDYLSVVLNQLCVLHEKTPVSDRVTKCCTESLVNRRPCFSALEVDETYVPKEFNAETFTFHADICTLSEKERQIKKQTALVELVKHKPKATKEQLKAVMDDFAAFVEKCCKADDKETCFAEEGKKLVAASQAALGL

SEQ ID NO: 98 - protein, 652 aa, Artificial Sequence
  Fusion protein
MKWVTFISLLFLFSSAYSCAEWSTAWGPCSTTCGLGMATRVSNQNRFCRLETQRRLCLSRPCEAAAKDAHKSEVAHRFKDLGEENFKALVLIAFAQYLQQCPFEDHVKLVNEVTEFAKTCVADESAENCDKSLHTLFGDKLCTVATLRETYGEMADCCAKQEPERNECFLQHKDDNPNLPRLVRPEVDVMCTAFHDNEETFLKKYLYEIARRHPYFYAPELLFFAKRYKAAFTECCQAADKAACLLPKLDELRDEGKASSAKQRLKCASLQKFGERAFKAWAVARLSQRFPKAEFAEVSKLVTDLTKVHTECCHGDLLECADDRADLAKYICENQDSISSKLKECCEKPLLEKSHCIAEVENDEMPADLPSLAADFVESKDVCKNYAEAKDVFLGMFLYEYARRHPDYSVVLLLRLAKTYETTLEKCCAAADPHECYAKVFDEFKPLVEEPQNLIKQNCELFEQLGEYKFQNALLVRYTKKVPQVSTPTLVEVSRNLGKVGSKCCKHPEAKRMPCAEDYLSVVLNQLCVLHEKTPVSDRVTKCCTESLVNRRPCFSALEVDETYVPKEFNAETFTFHADICTLSEKERQIKKQTALVELVKHKPKATKEQLKAVMDDFAAFVEKCCKADDKETCFAEEGKKLVAASQAALGL

SEQ ID NO: 99 - DNA, 1965 bp, Artificial Sequence
  Fusion protein
gccaccatgaaatgggtcacctttatctccctgctgttcctgttctcctccgcctactcttgcgccgagtggtctacagcttggggcccttgttctaccacctgtggcctcggcatggccaccagagtgtccaaccagaacagattctgccggctggaaacccagcggagactgtgcttgtctagaccttgcgaggccgctgccaaggacgctcataagtctgaggtggcccaccggttcaaggacctgggcgaagagaacttcaaggccctggtgctgatcgccttcgctcagtacttgcagcagtgccccttcgaggaccacgtgaagctggtcaacgaagtgaccgagttcgccaagacctgcgtggccgatgagtctgccgagaactgcgacaagtctctgcacaccctgttcggcgacaagctgtgtaccgtggctaccctgagagaaacctacggcgagatggccgactgctgcgctaagcaagagcccgagagaaacgagtgcttcctgcagcacaaggacgacaaccctaacctgcctagactcgtgcggcctgaggtggacgtgatgtgtaccgccttccacgacaacgaggaaaccttcctgaagaagtacctgtacgagatcgccagacggcacccctacttttacgcccctgagctgctgttcttcgccaagcggtacaaggccgccttcaccgagtgttgtcaggccgctgataaggccgcttgcctgctgcctaaactggacgagctgagagatgaaggcaaggcctccagcgccaagcagagactgaagtgtgccagcctgcagaagttcggcgagagagcctttaaggcctgggccgtcgctagactgtcccagagatttcccaaggccgagtttgccgaggtgtccaagctggttaccgacctgaccaaggtgcacaccgaatgctgtcacggcgacctgctggaatgcgccgatgatagagccgatctggccaagtacatctgcgagaaccaggactccatctcctccaagctgaaagagtgctgcgagaagcctctgctggaaaagtcccactgtatcgccgaggtggaaaacgacgagatgcctgccgatctgccttctctggccgccgacttcgtggaatctaaggacgtgtgcaagaactacgccgaggctaaggatgtgttcctgggcatgtttctgtacgagtacgctcggcggcaccccgactattctgttgtgctgctgctgagactggctaagacctacgagacaaccctcgagaagtgctgtgccgccgctgatcctcacgagtgttacgccaaggtgttcgacgagttcaagccactggtggaagaaccccagaacctgatcaagcagaattgcgagctgttcgagcagctgggcgagtacaagttccagaacgccctgctcgtgcggtacaccaagaaagtgccccaggtgtccacacctacactggttgaggtgtcccggaacctgggcaaagtgggctctaagtgctgcaagcaccccgaggccaagagaatgccttgtgccgaggactacctgtccgtggtgctgaaccagctgtgcgtgctgcacgaaaagacccctgtgtccgacagagtgaccaagtgctgtaccgagagcctggtcaacagacggccttgcttctctgccctggaagtggacgagacatacgtgcccaaagagttcaacgccgagacattcaccttccacgccgacatctgcaccctgtccgagaaagagcggcagatcaagaaacagaccgctctggtggaactggtcaagcacaagcccaaggccaccaaagaacagctgaaggccgtgatggacgacttcgccgcctttgtggaaaagtgttgcaaggccgacgacaaagagacatgcttcgccgaagagggcaagaaactggtggccgcttctcaggctgctctgggactttaa

SEQ ID NO: 100 - DNA, 2038 bp, Artificial Sequence
  Fusion protein
ggggacaagtttgtacaaaaaagcaggctatggtaccgccaccatgaaatgggtcacctttatctccctgctgttcctgttctcctccgcctactcttgcgccgagtggtctacagcttggggcccttgttctaccacctgtggcctcggcatggccaccagagtgtccaaccagaacagattctgccggctggaaacccagcggagactgtgcttgtctagaccttgcgaggccgctgccaaggacgctcataagtctgaggtggcccaccggttcaaggacctgggcgaagagaacttcaaggccctggtgctgatcgccttcgctcagtacttgcagcagtgccccttcgaggaccacgtgaagctggtcaacgaagtgaccgagttcgccaagacctgcgtggccgatgagtctgccgagaactgcgacaagtctctgcacaccctgttcggcgacaagctgtgtaccgtggctaccctgagagaaacctacggcgagatggccgactgctgcgctaagcaagagcccgagagaaacgagtgcttcctgcagcacaaggacgacaaccctaacctgcctagactcgtgcggcctgaggtggacgtgatgtgtaccgccttccacgacaacgaggaaaccttcctgaagaagtacctgtacgagatcgccagacggcacccctacttttacgcccctgagctgctgttcttcgccaagcggtacaaggccgccttcaccgagtgttgtcaggccgctgataaggccgcttgcctgctgcctaaactggacgagctgagagatgaaggcaaggcctccagcgccaagcagagactgaagtgtgccagcctgcagaagttcggcgagagagcctttaaggcctgggccgtcgctagactgtcccagagatttcccaaggccgagtttgccgaggtgtccaagctggttaccgacctgaccaaggtgcacaccgaatgctgtcacggcgacctgctggaatgcgccgatgatagagccgatctggccaagtacatctgcgagaaccaggactccatctcctccaagctgaaagagtgctgcgagaagcctctgctggaaaagtcccactgtatcgccgaggtggaaaacgacgagatgcctgccgatctgccttctctggccgccgacttcgtggaatctaaggacgtgtgcaagaactacgccgaggctaaggatgtgttcctgggcatgtttctgtacgagtacgctcggcggcaccccgactattctgttgtgctgctgctgagactggctaagacctacgagacaaccctcgagaagtgctgtgccgccgctgatcctcacgagtgttacgccaaggtgttcgacgagttcaagccactggtggaagaaccccagaacctgatcaagcagaattgcgagctgttcgagcagctgggcgagtacaagttccagaacgccctgctcgtgcggtacaccaagaaagtgccccaggtgtccacacctacactggttgaggtgtcccggaacctgggcaaagtgggctctaagtgctgcaagcaccccgaggccaagagaatgccttgtgccgaggactacctgtccgtggtgctgaaccagctgtgcgtgctgcacgaaaagacccctgtgtccgacagagtgaccaagtgctgtaccgagagcctggtcaacagacggccttgcttctctgccctggaagtggacgagacatacgtgcccaaagagttcaacgccgagacattcaccttccacgccgacatctgcaccctgtccgagaaagagcggcagatcaagaaacagaccgctctggtggaactggtcaagcacaagcccaaggccaccaaagaacagctgaaggccgtgatggacgacttcgccgcctttgtggaaaagtgttgcaaggccgacgacaaagagacatgcttcgccgaagagggcaagaaactggtggccgcttctcaggctgctctgggactttaatctagaaacccagctttcttgtacaaagtggtcccc

SEQ ID NO: 101 - protein, 582 aa, Homo sapiens
DAHKSEVAHRFKDLGEENFKALVLIAFAQYLQQCPFEDHVKLVNEVTEFAKTCVADESAENCDKSLHTLFGDKLCTVATLRETYGEMADCCAKQEPERNECFLQHKDDNPNLPRLVRPEVDVMCTAFHDNEETFLKKYLYEIARRHPYFYAPELLFFAKRYKAAFTECCQAADKAACLLPKLDELRDEGKASSAKQRLKCASLQKFGERAFKAWAVARLSQRFPKAEFAEVSKLVTDLTKVHTECCHGDLLECADDRADLAKYICENQDSISSKLKECCEKPLLEKSHCIAEVENDEMPADLPSLAADFVESKDVCKNYAEAKDVFLGMFLYEYARRHPDYSVVLLLRLAKTYETTLEKCCAAADPHECYAKVFDEFKPLVEEPQNLIKQNCELFEQLGEYKFQNALLVRYTKKVPQVSTPTLVEVSRNLGKVGSKCCKHPEAKRMPCAEDYLSVVLNQLCVLHEKTPVSDRVTKCCTESLVNRRPCFSALEVDETYVPKEFNAETFTFHADICTLSEKERQIKKQTALVELVKHKPKATKEQLKAVMDDFAAFVEKCCKADDKETCFAEEGKKLVAASQAA

SEQ ID NO: 102 - protein, 675 aa, Artificial Sequence
  Fusion protein
DAHKSEVAHRFKDLGEENFKALVLIAFAQYLQQCPFEDHVKLVNEVTEFAKTCVADESAENCDKSLHTLFGDKLCTVATLRETYGEMADCCAKQEPERNECFLQHKDDNPNLPRLVRPEVDVMCTAFHDNEETFLKKYLYEIARRHPYFYAPELLFFAKRYKAAFTECCQAADKAACLLPKLDELRDEGKASSAKQRLKCASLQKFGERAFKAWAVARLSQRFPKAEFAEVSKLVTDLTKVHTECCHGDLLECADDRADLAKYICENQDSISSKLKECCEKPLLEKSHCIAEVENDEMPADLPSLAADFVESKDVCKNYAEAKDVFLGMFLYEYARRHPDYSVVLLLRLAKTYETTLEKCCAAADPHECYAKVFDEFKPLVEEPQNLIKQNCELFEQLGEYKFQNALLVRYTKKVPQVSTPTLVEVSRNLGKVGSKCCKHPEAKRMPCAEDYLSVVLNQLCVLHEKTPVSDRVTKCCTESLVNRRPCFSALEVDETYVPKEFNAETFTFHADICTLSEKERQIKKQTALVELVKHKPKATKEQLKAVMDDFAAFVEKCCKADDKETCFAEEGKKLVAASQAAEAAAKEAAAKEAAAKEAAAKEAAAKEAAAKEAAAKEAAAKCAEWSTAWGPCSTTCGLGMATRVSNQNRFCRLETQRRLCLSRPCPPSRGRSPQ

SEQ ID NO: 103 - protein, 693 aa, Artificial Sequence
  Fusion protein
MKWVTFISLLFLFSSAYSDAHKSEVAHRFKDLGEENFKALVLIAFAQYLQQCPFEDHVKLVNEVTEFAKTCVADESAENCDKSLHTLFGDKLCTVATLRETYGEMADCCAKQEPERNECFLQHKDDNPNLPRLVRPEVDVMCTAFHDNEETFLKKYLYEIARRHPYFYAPELLFFAKRYKAAFTECCQAADKAACLLPKLDELRDEGKASSAKQRLKCASLQKFGERAFKAWAVARLSQRFPKAEFAEVSKLVTDLTKVHTECCHGDLLECADDRADLAKYICENQDSISSKLKECCEKPLLEKSHCIAEVENDEMPADLPSLAADFVESKDVCKNYAEAKDVFLGMFLYEYARRHPDYSVVLLLRLAKTYETTLEKCCAAADPHECYAKVFDEFKPLVEEPQNLIKQNCELFEQLGEYKFQNALLVRYTKKVPQVSTPTLVEVSRNLGKVGSKCCKHPEAKRMPCAEDYLSVVLNQLCVLHEKTPVSDRVTKCCTESLVNRRPCFSALEVDETYVPKEFNAETFTFHADICTLSEKERQIKKQTALVELVKHKPKATKEQLKAVMDDFAAFVEKCCKADDKETCFAEEGKKLVAASQAAEAAAKEAAAKEAAAKEAAAKEAAAKEAAAKEAAAKEAAAKCAEWSTAWGPCSTTCGLGMATRVSNQNRFCRLETQRRLCLSRPCPPSRGRSPQ

SEQ ID NO: 104 - DNA, 2088 bp, Artificial Sequence
  Fusion protein
gccaccatgaaatgggtcacctttatctccctgctgttcctgttctcctccgcctactctgacgcccacaagtctgaggtggcccacagattcaaggacctgggcgaagagaacttcaaggccctggtgctgatcgccttcgctcagtacttgcagcagtgccccttcgaggaccacgtgaagctggtcaacgaagtgaccgagttcgccaagacctgcgtggccgatgagtctgccgagaactgcgacaagtctctgcacaccctgttcggcgacaagctgtgtaccgtggctaccctgagagaaacctacggcgagatggccgactgctgcgctaagcaagagcccgagagaaacgagtgcttcctgcagcacaaggacgacaaccctaacctgcctagactcgtgcggcctgaggtggacgtgatgtgtaccgccttccacgacaacgaggaaaccttcctgaagaagtacctgtacgagatcgccagacggcacccctacttttacgcccctgagctgctgttcttcgccaagcggtacaaggccgccttcaccgagtgttgtcaggccgctgataaggccgcttgcctgctgcctaaactggacgagctgagagatgaaggcaaggcctccagcgccaagcagagactgaagtgtgccagcctgcagaagttcggcgagagagcctttaaggcctgggccgtcgctagactgtcccagagatttcccaaggccgagtttgccgaggtgtccaagctggttaccgacctgaccaaggtgcacaccgaatgctgtcacggcgacctgctggaatgcgccgatgatagagccgatctggccaagtacatctgcgagaaccaggactccatctcctccaagctgaaagagtgctgcgagaagcctctgctggaaaagtcccactgtatcgccgaggtggaaaacgacgagatgcctgccgatctgccttctctggccgccgacttcgtggaatctaaggacgtgtgcaagaactacgccgaggccaaggatgtgttcctgggcatgtttctgtacgagtacgctcggcggcaccccgactattctgttgtgctgctgctgagactggctaagacctacgagacaaccctcgagaagtgctgtgccgccgctgatcctcacgagtgttacgccaaggtgttcgacgagttcaagccactggtggaagaaccccagaacctgatcaagcagaattgcgagctgttcgagcagctgggcgagtacaagttccagaacgccctgctcgtgcggtacaccaagaaagtgccccaggtgtccacacctacactggttgaggtgtcccggaacctgggcaaagtgggctctaagtgctgcaagcaccctgaggccaagagaatgccttgcgccgaggactacctgtccgtggtgctgaatcagctgtgcgtgctgcacgaaaagacccctgtgtccgacagagtgaccaagtgctgtaccgagagcctggtcaacagacggccttgcttctctgccctggaagtggacgagacatacgtgcccaaagagttcaacgccgagacattcaccttccacgccgacatctgcaccctgtccgagaaagagcggcagatcaagaaacagaccgctctggtggaactggtcaagcacaagcccaaggccaccaaagaacagctgaaggccgtgatggacgacttcgccgcctttgtggaaaagtgttgcaaggccgacgacaaagagacatgcttcgccgaagagggcaagaaactggtggccgcttctcaggctgctgaggccgctgctaaagaggctgccgctaaagaagccgcagccaaagaggcagctgcaaaagaagctgctgcaaaagaggcagccgccaaagaggccgctgctaaagaagcagccgccaagtgtgctgagtggtctacagcttggggcccctgctctacaacctgtggactcggcatggccaccagagtgtctaaccagaacagattctgccggctggaaacccagcggagactgtgcctgtctagaccctgtcctcctagcagaggcagatcccctcagtga

SEQ ID NO: 105 - DNA, 2161 bp, Artificial Sequence
  Fusion protein
ggggacaagtttgtacaaaaaagcaggctatggtaccgccaccatgaaatgggtcacctttatctccctgctgttcctgttctcctccgcctactctgacgcccacaagtctgaggtggcccacagattcaaggacctgggcgaagagaacttcaaggccctggtgctgatcgccttcgctcagtacttgcagcagtgccccttcgaggaccacgtgaagctggtcaacgaagtgaccgagttcgccaagacctgcgtggccgatgagtctgccgagaactgcgacaagtctctgcacaccctgttcggcgacaagctgtgtaccgtggctaccctgagagaaacctacggcgagatggccgactgctgcgctaagcaagagcccgagagaaacgagtgcttcctgcagcacaaggacgacaaccctaacctgcctagactcgtgcggcctgaggtggacgtgatgtgtaccgccttccacgacaacgaggaaaccttcctgaagaagtacctgtacgagatcgccagacggcacccctacttttacgcccctgagctgctgttcttcgccaagcggtacaaggccgccttcaccgagtgttgtcaggccgctgataaggccgcttgcctgctgcctaaactggacgagctgagagatgaaggcaaggcctccagcgccaagcagagactgaagtgtgccagcctgcagaagttcggcgagagagcctttaaggcctgggccgtcgctagactgtcccagagatttcccaaggccgagtttgccgaggtgtccaagctggttaccgacctgaccaaggtgcacaccgaatgctgtcacggcgacctgctggaatgcgccgatgatagagccgatctggccaagtacatctgcgagaaccaggactccatctcctccaagctgaaagagtgctgcgagaagcctctgctggaaaagtcccactgtatcgccgaggtggaaaacgacgagatgcctgccgatctgccttctctggccgccgacttcgtggaatctaaggacgtgtgcaagaactacgccgaggccaaggatgtgttcctgggcatgtttctgtacgagtacgctcggcggcaccccgactattctgttgtgctgctgctgagactggctaagacctacgagacaaccctcgagaagtgctgtgccgccgctgatcctcacgagtgttacgccaaggtgttcgacgagttcaagccactggtggaagaaccccagaacctgatcaagcagaattgcgagctgttcgagcagctgggcgagtacaagttccagaacgccctgctcgtgcggtacaccaagaaagtgccccaggtgtccacacctacactggttgaggtgtcccggaacctgggcaaagtgggctctaagtgctgcaagcaccctgaggccaagagaatgccttgcgccgaggactacctgtccgtggtgctgaatcagctgtgcgtgctgcacgaaaagacccctgtgtccgacagagtgaccaagtgctgtaccgagagcctggtcaacagacggccttgcttctctgccctggaagtggacgagacatacgtgcccaaagagttcaacgccgagacattcaccttccacgccgacatctgcaccctgtccgagaaagagcggcagatcaagaaacagaccgctctggtggaactggtcaagcacaagcccaaggccaccaaagaacagctgaaggccgtgatggacgacttcgccgcctttgtggaaaagtgttgcaaggccgacgacaaagagacatgcttcgccgaagagggcaagaaactggtggccgcttctcaggctgctgaggccgctgctaaagaggctgccgctaaagaagccgcagccaaagaggcagctgcaaaagaagctgctgcaaaagaggcagccgccaaagaggccgctgctaaagaagcagccgccaagtgtgctgagtggtctacagcttggggcccctgctctacaacctgtggactcggcatggccaccagagtgtctaaccagaacagattctgccggctggaaacccagcggagactgtgcctgtctagaccctgtcctcctagcagaggcagatcccctcagtgatctagaaacccagctttcttgtacaaagtggtcccc

SEQ ID NO: 106 - protein, 634 aa, Artificial Sequence
  Fusion protein
CAEQTTEWTACSKSCGMGFSTRVTNRNRQCEMLKQTRLCMVRPCEAAAKDAHKSEVAHRFKDLGEENFKALVLIAFAQYLQQCPFEDHVKLVNEVTEFAKTCVADESAENCDKSLHTLFGDKLCTVATLRETYGEMADCCAKQEPERNECFLQHKDDNPNLPRLVRPEVDVMCTAFHDNEETFLKKYLYEIARRHPYFYAPELLFFAKRYKAAFTECCQAADKAACLLPKLDELRDEGKASSAKQRLKCASLQKFGERAFKAWAVARLSQRFPKAEFAEVSKLVTDLTKVHTECCHGDLLECADDRADLAKYICENQDSISSKLKECCEKPLLEKSHCIAEVENDEMPADLPSLAADFVESKDVCKNYAEAKDVFLGMFLYEYARRHPDYSVVLLLRLAKTYETTLEKCCAAADPHECYAKVFDEFKPLVEEPQNLIKQNCELFEQLGEYKFQNALLVRYTKKVPQVSTPTLVEVSRNLGKVGSKCCKHPEAKRMPCAEDYLSVVLNQLCVLHEKTPVSDRVTKCCTESLVNRRPCFSALEVDETYVPKEFNAETFTFHADICTLSEKERQIKKQTALVELVKHKPKATKEQLKAVMDDFAAFVEKCCKADDKETCFAEEGKKLVAASQAALGL

SEQ ID NO: 107 - protein, 652 aa, Artificial Sequence
  Fusion protein
MKWVTFISLLFLFSSAYSCAEQTTEWTACSKSCGMGFSTRVTNRNRQCEMLKQTRLCMVRPCEAAAKDAHKSEVAHRFKDLGEENFKALVLIAFAQYLQQCPFEDHVKLVNEVTEFAKTCVADESAENCDKSLHTLFGDKLCTVATLRETYGEMADCCAKQEPERNECFLQHKDDNPNLPRLVRPEVDVMCTAFHDNEETFLKKYLYEIARRHPYFYAPELLFFAKRYKAAFTECCQAADKAACLLPKLDELRDEGKASSAKQRLKCASLQKFGERAFKAWAVARLSQRFPKAEFAEVSKLVTDLTKVHTECCHGDLLECADDRADLAKYICENQDSISSKLKECCEKPLLEKSHCIAEVENDEMPADLPSLAADFVESKDVCKNYAEAKDVFLGMFLYEYARRHPDYSVVLLLRLAKTYETTLEKCCAAADPHECYAKVFDEFKPLVEEPQNLIKQNCELFEQLGEYKFQNALLVRYTKKVPQVSTPTLVEVSRNLGKVGSKCCKHPEAKRMPCAEDYLSVVLNQLCVLHEKTPVSDRVTKCCTESLVNRRPCFSALEVDETYVPKEFNAETFTFHADICTLSEKERQIKKQTALVELVKHKPKATKEQLKAVMDDFAAFVEKCCKADDKETCFAEEGKKLVAASQAALGL

SEQ ID NO: 108 - DNA, 1965 bp, Artificial Sequence
  Fusion protein
gccaccatgaaatgggtcacctttatctccctgctgttcctgttctcctccgcctactcttgtgccgagcagaccacagagtggaccgcctgctctaagtcttgcggcatgggcttctccaccagagtgaccaaccggaacagacagtgcgagatgctgaagcagacccggctgtgtatggttcgaccttgcgaggccgctgccaaggatgctcataagtctgaggtggcccaccggttcaaggacctgggcgaagagaacttcaaggccctggtgctgatcgccttcgctcagtacttgcagcagtgccccttcgaggaccacgtgaagctggtcaacgaagtgaccgagttcgccaagacctgcgtggccgatgagtctgccgagaactgcgacaagtctctgcacaccctgttcggcgacaagctgtgtaccgtggctaccctgagagaaacctacggcgagatggccgactgctgcgctaagcaagagcccgagagaaacgagtgcttcctgcagcacaaggacgacaaccctaacctgcctagactcgtgcggcctgaggtggacgtgatgtgtaccgccttccacgacaacgaggaaaccttcctgaagaagtacctgtacgagatcgccagacggcacccctacttttacgcccctgagctgctgttcttcgccaagcggtacaaggccgccttcaccgagtgttgtcaggccgctgataaggccgcttgcctgctgcctaaactggacgagctgagagatgaaggcaaggcctccagcgccaagcagagactgaagtgtgccagcctgcagaagttcggcgagagagcctttaaggcctgggccgtcgctagactgtcccagagatttcccaaggccgagtttgccgaggtgtccaagctggttaccgacctgaccaaggtgcacaccgaatgctgtcacggcgacctgctggaatgcgccgatgatagagccgatctggccaagtacatctgcgagaaccaggactccatctcctccaagctgaaagagtgctgcgagaagcctctgctggaaaagtcccactgtatcgccgaggtggaaaacgacgagatgcctgccgatctgccttctctggccgccgacttcgtggaatctaaggacgtgtgcaagaactacgccgaggctaaggatgtgttcctgggcatgtttctgtacgagtacgctcggcggcaccccgattatagtgtggtgctgctgctgagactggctaagacctacgagacaaccctcgagaagtgctgtgccgccgctgatcctcacgagtgttacgccaaggtgttcgacgagttcaagccactggtggaagaaccccagaacctgatcaagcagaattgcgagctgttcgagcagctgggcgagtacaagttccagaacgccctgctcgtgcggtacaccaagaaagtgccccaggtgtccacacctacactggttgaggtgtcccggaacctgggcaaagtgggctctaagtgctgcaagcaccccgaggccaagagaatgccttgcgccgaggattacctgtccgtggtgctgaaccagctgtgcgtgctgcacgaaaagacccctgtgtccgaccgcgtgaccaagtgctgtacagagtccctggtcaacagacggccctgcttctctgccctggaagtggacgagacatacgtgcccaaagagttcaacgccgagacattcaccttccacgccgacatctgcaccctgtccgagaaagagcggcagatcaagaaacagaccgctctggtcgaactggtcaagcacaagcccaaggccaccaaagaacagctgaaggccgtgatggacgacttcgccgcctttgtggaaaagtgttgcaaggccgacgacaaagagacatgcttcgccgaagagggcaagaaactggtggccgcttctcaggctgctctgggactttaa

SEQ ID NO: 109 - DNA, 2038 bp, Artificial Sequence
  Fusion protein
ggggacaagtttgtacaaaaaagcaggctatggtaccgccaccatgaaatgggtcacctttatctccctgctgttcctgttctcctccgcctactcttgtgccgagcagaccacagagtggaccgcctgctctaagtcttgcggcatgggcttctccaccagagtgaccaaccggaacagacagtgcgagatgctgaagcagacccggctgtgtatggttcgaccttgcgaggccgctgccaaggatgctcataagtctgaggtggcccaccggttcaaggacctgggcgaagagaacttcaaggccctggtgctgatcgccttcgctcagtacttgcagcagtgccccttcgaggaccacgtgaagctggtcaacgaagtgaccgagttcgccaagacctgcgtggccgatgagtctgccgagaactgcgacaagtctctgcacaccctgttcggcgacaagctgtgtaccgtggctaccctgagagaaacctacggcgagatggccgactgctgcgctaagcaagagcccgagagaaacgagtgcttcctgcagcacaaggacgacaaccctaacctgcctagactcgtgcggcctgaggtggacgtgatgtgtaccgccttccacgacaacgaggaaaccttcctgaagaagtacctgtacgagatcgccagacggcacccctacttttacgcccctgagctgctgttcttcgccaagcggtacaaggccgccttcaccgagtgttgtcaggccgctgataaggccgcttgcctgctgcctaaactggacgagctgagagatgaaggcaaggcctccagcgccaagcagagactgaagtgtgccagcctgcagaagttcggcgagagagcctttaaggcctgggccgtcgctagactgtcccagagatttcccaaggccgagtttgccgaggtgtccaagctggttaccgacctgaccaaggtgcacaccgaatgctgtcacggcgacctgctggaatgcgccgatgatagagccgatctggccaagtacatctgcgagaaccaggactccatctcctccaagctgaaagagtgctgcgagaagcctctgctggaaaagtcccactgtatcgccgaggtggaaaacgacgagatgcctgccgatctgccttctctggccgccgacttcgtggaatctaaggacgtgtgcaagaactacgccgaggctaaggatgtgttcctgggcatgtttctgtacgagtacgctcggcggcaccccgattatagtgtggtgctgctgctgagactggctaagacctacgagacaaccctcgagaagtgctgtgccgccgctgatcctcacgagtgttacgccaaggtgttcgacgagttcaagccactggtggaagaaccccagaacctgatcaagcagaattgcgagctgttcgagcagctgggcgagtacaagttccagaacgccctgctcgtgcggtacaccaagaaagtgccccaggtgtccacacctacactggttgaggtgtcccggaacctgggcaaagtgggctctaagtgctgcaagcaccccgaggccaagagaatgccttgcgccgaggattacctgtccgtggtgctgaaccagctgtgcgtgctgcacgaaaagacccctgtgtccgaccgcgtgaccaagtgctgtacagagtccctggtcaacagacggccctgcttctctgccctggaagtggacgagacatacgtgcccaaagagttcaacgccgagacattcaccttccacgccgacatctgcaccctgtccgagaaagagcggcagatcaagaaacagaccgctctggtcgaactggtcaagcacaagcccaaggccaccaaagaacagctgaaggccgtgatggacgacttcgccgcctttgtggaaaagtgttgcaaggccgacgacaaagagacatgcttcgccgaagagggcaagaaactggtggccgcttctcaggctgctctgggactttaatctagaaacccagctttcttgtacaaagtggtcccc

SEQ ID NO: 110 - protein, 669 aa, Artificial Sequence
  Fusion protein
CAEQTTEWTACSKSCGMGFSTRVTNRNRQCEMLKQTRLCMVRPCEAAAKEAAAKEAAAKEAAAKEAAAKEAAAKEAAAKEAAAKDAHKSEVAHRFKDLGEENFKALVLIAFAQYLQQCPFEDHVKLVNEVTEFAKTCVADESAENCDKSLHTLFGDKLCTVATLRETYGEMADCCAKQEPERNECFLQHKDDNPNLPRLVRPEVDVMCTAFHDNEETFLKKYLYEIARRHPYFYAPELLFFAKRYKAAFTECCQAADKAACLLPKLDELRDEGKASSAKQRLKCASLQKFGERAFKAWAVARLSQRFPKAEFAEVSKLVTDLTKVHTECCHGDLLECADDRADLAKYICENQDSISSKLKECCEKPLLEKSHCIAEVENDEMPADLPSLAADFVESKDVCKNYAEAKDVFLGMFLYEYARRHPDYSVVLLLRLAKTYETTLEKCCAAADPHECYAKVFDEFKPLVEEPQNLIKQNCELFEQLGEYKFQNALLVRYTKKVPQVSTPTLVEVSRNLGKVGSKCCKHPEAKRMPCAEDYLSVVLNQLCVLHEKTPVSDRVTKCCTESLVNRRPCFSALEVDETYVPKEFNAETFTFHADICTLSEKERQIKKQTALVELVKHKPKATKEQLKAVMDDFAAFVEKCCKADDKETCFAEEGKKLVAASQAALGL

SEQ ID NO: 111 - protein, 687 aa, Artificial Sequence
  Fusion protein
MKWVTFISLLFLFSSAYSCAEQTTEWTACSKSCGMGFSTRVTNRNRQCEMLKQTRLCMVRPCEAAAKEAAAKEAAAKEAAAKEAAAKEAAAKEAAAKEAAAKDAHKSEVAHRFKDLGEENFKALVLIAFAQYLQQCPFEDHVKLVNEVTEFAKTCVADESAENCDKSLHTLFGDKLCTVATLRETYGEMADCCAKQEPERNECFLQHKDDNPNLPRLVRPEVDVMCTAFHDNEETFLKKYLYEIARRHPYFYAPELLFFAKRYKAAFTECCQAADKAACLLPKLDELRDEGKASSAKQRLKCASLQKFGERAFKAWAVARLSQRFPKAEFAEVSKLVTDLTKVHTECCHGDLLECADDRADLAKYICENQDSISSKLKECCEKPLLEKSHCIAEVENDEMPADLPSLAADFVESKDVCKNYAEAKDVFLGMFLYEYARRHPDYSVVLLLRLAKTYETTLEKCCAAADPHECYAKVFDEFKPLVEEPQNLIKQNCELFEQLGEYKFQNALLVRYTKKVPQVSTPTLVEVSRNLGKVGSKCCKHPEAKRMPCAEDYLSVVLNQLCVLHEKTPVSDRVTKCCTESLVNRRPCFSALEVDETYVPKEFNAETFTFHADICTLSEKERQIKKQTALVELVKHKPKATKEQLKAVMDDFAAFVEKCCKADDKETCFAEEGKKLVAASQAALGL

SEQ ID NO: 112 - DNA, 2070 bp, Artificial Sequence
  Fusion protein
gccaccatgaaatgggtcacctttatctccctgctgttcctgttctcctccgcctactcttgtgccgagcagaccacagagtggaccgcctgctctaagtcttgcggcatgggcttctccaccagagtgaccaaccggaacagacagtgcgagatgctgaagcagacccggctgtgtatggttcgaccttgcgaggccgctgccaaagaggctgctgctaaagaagccgccgcaaaagaggcagcagcaaaagaggctgccgccaaagaggccgcagccaaagaagcagcagctaaagaggccgctgctaaggacgcccacaagtctgaagtggcccaccggtttaaggacctgggcgaagagaacttcaaggccctggtgctgatcgccttcgctcagtacttgcagcagtgccccttcgaggaccacgtgaagctggtcaacgaagtgaccgagttcgccaagacctgcgtggccgatgagtctgccgagaactgcgacaagtctctgcacaccctgttcggcgacaagctgtgtaccgtggctaccctgagagaaacctacggcgagatggccgactgctgcgctaagcaagagcccgagagaaacgagtgcttcctgcagcacaaggacgacaaccctaacctgcctagactcgtgcggcctgaggtggacgtgatgtgtaccgccttccacgacaacgaggaaaccttcctgaagaagtacctgtacgagatcgccagacggcacccctacttttacgcccctgagctgctgtttttcgccaagcggtacaaggccgccttcaccgagtgttgtcaggccgccgataaggccgcttgtctgctgcctaaactggacgagctgcgcgacgaaggcaaggcctcttctgctaagcagcggctgaagtgcgccagcctgcagaagtttggcgagagagccttcaaggcttgggccgtcgctagactgtcccagagatttcccaaggccgagtttgccgaggtgtccaagctggttaccgacctgaccaaggtgcacaccgaatgctgtcacggcgacctgctggaatgcgccgatgatagagccgatctggccaagtacatctgcgagaaccaggactccatctcctccaagctgaaagagtgctgcgagaagcctctgctggaaaagtcccactgtatcgccgaggtggaaaacgacgagatgcctgccgatctgccttctctggccgccgacttcgtggaatctaaggacgtgtgcaagaactacgccgaggccaaggatgtgttcctgggcatgtttctgtacgagtacgctcggcggcaccccgattatagtgtggtgctgctgctgagactggctaagacctacgagacaaccctcgagaagtgctgtgccgccgctgatcctcacgagtgttacgccaaggtgttcgacgagttcaagccactggtggaagaaccccagaacctgatcaagcagaattgcgagctgttcgagcagctgggcgagtacaagttccagaacgccctgctcgtgcggtacaccaagaaagtgccccaggtgtccacacctacactggttgaggtgtcccggaacctgggcaaagtgggctctaagtgctgcaagcaccctgaggccaagagaatgccttgcgccgaggactacctgtccgtggtgctgaatcagctgtgcgtgctgcacgaaaagacccctgtgtccgaccgcgtgaccaagtgctgtacagagtccctggtcaacagacggccctgcttctctgccctggaagtggacgagacatacgtgcccaaagagttcaacgccgagacattcaccttccacgccgacatctgcaccctgtccgagaaagagcggcagatcaagaaacagaccgctctggtcgagctggttaagcacaagcccaaggccaccaaagaacagctgaaggccgtgatggacgacttcgccgcctttgtggaaaagtgttgcaaggccgacgacaaagagacatgcttcgccgaagagggcaagaaactggtggccgcttctcaggctgctctgggactttaa

SEQ ID NO: 113 - DNA, 2143 bp, Artificial Sequence
  Fusion protein
ggggacaagtttgtacaaaaaagcaggctatggtaccgccaccatgaaatgggtcacctttatctccctgctgttcctgttctcctccgcctactcttgtgccgagcagaccacagagtggaccgcctgctctaagtcttgcggcatgggcttctccaccagagtgaccaaccggaacagacagtgcgagatgctgaagcagacccggctgtgtatggttcgaccttgcgaggccgctgccaaagaggctgctgctaaagaagccgccgcaaaagaggcagcagcaaaagaggctgccgccaaagaggccgcagccaaagaagcagcagctaaagaggccgctgctaaggacgcccacaagtctgaagtggcccaccggtttaaggacctgggcgaagagaacttcaaggccctggtgctgatcgccttcgctcagtacttgcagcagtgccccttcgaggaccacgtgaagctggtcaacgaagtgaccgagttcgccaagacctgcgtggccgatgagtctgccgagaactgcgacaagtctctgcacaccctgttcggcgacaagctgtgtaccgtggctaccctgagagaaacctacggcgagatggccgactgctgcgctaagcaagagcccgagagaaacgagtgcttcctgcagcacaaggacgacaaccctaacctgcctagactcgtgcggcctgaggtggacgtgatgtgtaccgccttccacgacaacgaggaaaccttcctgaagaagtacctgtacgagatcgccagacggcacccctacttttacgcccctgagctgctgtttttcgccaagcggtacaaggccgccttcaccgagtgttgtcaggccgccgataaggccgcttgtctgctgcctaaactggacgagctgcgcgacgaaggcaaggcctcttctgctaagcagcggctgaagtgcgccagcctgcagaagtttggcgagagagccttcaaggcttgggccgtcgctagactgtcccagagatttcccaaggccgagtttgccgaggtgtccaagctggttaccgacctgaccaaggtgcacaccgaatgctgtcacggcgacctgctggaatgcgccgatgatagagccgatctggccaagtacatctgcgagaaccaggactccatctcctccaagctgaaagagtgctgcgagaagcctctgctggaaaagtcccactgtatcgccgaggtggaaaacgacgagatgcctgccgatctgccttctctggccgccgacttcgtggaatctaaggacgtgtgcaagaactacgccgaggccaaggatgtgttcctgggcatgtttctgtacgagtacgctcggcggcaccccgattatagtgtggtgctgctgctgagactggctaagacctacgagacaaccctcgagaagtgctgtgccgccgctgatcctcacgagtgttacgccaaggtgttcgacgagttcaagccactggtggaagaaccccagaacctgatcaagcagaattgcgagctgttcgagcagctgggcgagtacaagttccagaacgccctgctcgtgcggtacaccaagaaagtgccccaggtgtccacacctacactggttgaggtgtcccggaacctgggcaaagtgggctctaagtgctgcaagcaccctgaggccaagagaatgccttgcgccgaggactacctgtccgtggtgctgaatcagctgtgcgtgctgcacgaaaagacccctgtgtccgaccgcgtgaccaagtgctgtacagagtccctggtcaacagacggccctgcttctctgccctggaagtggacgagacatacgtgcccaaagagttcaacgccgagacattcaccttccacgccgacatctgcaccctgtccgagaaagagcggcagatcaagaaacagaccgctctggtcgagctggttaagcacaagcccaaggccaccaaagaacagctgaaggccgtgatggacgacttcgccgcctttgtggaaaagtgttgcaaggccgacgacaaagagacatgcttcgccgaagagggcaagaaactggtggccgcttctcaggctgctctgggactttaatctagaaacccagctttcttgtacaaagtggtcccc

SEQ ID NO: 114 - protein, 484 aa, Artificial Sequence
  Fusion protein
MKWVTFISLLFLFSSAYSGHHHHHHGSEIGTGFPFDPHYVEVLGERMHYVDVGPRDGTPVLFLHGNPTSSYVWRNIIPHVAPTHRCIAPDLIGMGKSDKPDLGYFFDDHVRFMDAFIEALGLEEVVLVIHDWGSALGFHWAKRNPERVKGIAFMEFIRPIPTWDEWPEFARETFQAFRTTDVGRKLIIDQNVFIEGTLPMGVVRPLTEVEMDHYREPFLNPVDREPLWRFPNELPIAGEPANIVALVEEYMDWLHQSPVPKLLFWGTPGVLIPPAEAARLAKSLPNCKAVDIGPGLNLLQEDNPDLIGSEIARWLSTLEISGLQDSEVNQEAKPEVKPEVKPETHINLKVSDGSSEIFFKIKKTTPLRRLMEAFAKRQGKEMDSLTFLYDGIEIQADQTPEDLDMEDNDIIEAHREQIGGSGGSGGSGGSGGSSGGGSSGCAEQTTEWTACSKSCGMGFSTRVTNRNRQCEMLKQTRLCMVRPC

SEQ ID NO: 115 - protein, 13 aa, Artificial Sequence
  part of recombinant protein
PPSRGRSPQNSAF

SEQ ID NO: 116 - protein, 8 aa, Artificial Sequence
  part of recombinant protein
GQPVYSSL

SEQ ID NO: 117 - protein, 7 aa, Artificial Sequence
  part of recombinant protein
EADLEEN

SEQ ID NO: 118 - protein, 9 aa, Artificial Sequence
  part of recombinant protein
EQQPEQPTD

SEQ ID NO: 119 - protein, 8 aa, Artificial Sequence
  part of recombinant protein
DVDIHTLI

SEQ ID NO: 120 - protein, 11 aa, Artificial Sequence
  part of recombinant protein
DSNILKTIKIP

SEQ ID NO: 121 - protein, 5 aa, Artificial Sequence
  Linker
GGGGS